European Patent Application EP 4 130 027 A1, published February 8, 2023. Title: Novel immunostimulating IL-2 analogs. Applicant: HANMI PHARM. CO., LTD. The sequence listing filed with the application follows.

SEQUENCE LISTING (417 sequences)

SEQ ID NO: 1 - protein, 133 aa, homo sapiens [sequence omitted]

SEQ ID NO: 2 - protein, 132 aa, Artificial Sequence
  IL-2 analog 1
PTSSSTKKTQLQLEHLLLDLQMILNGINNYKNPKLTRMLTFKFYMPKKATELKHLQCLEEELKPLEEVLNLAQSKNFHLRPRDLISNINVIVLELKGSETTFMCEYADETATIVEFLNRWITFSQSIISTLT

SEQ ID NO: 3 - protein, 132 aa, Artificial Sequence
  IL-2 analog 2
PTSSSTKKTQLQLEHLLLDLQMILNGINNYKNPKLTRMLTFKFYMPKKATELKHLQCLEEELKPLEEVLNLAQSKNFHLRPRDLICNINVIVLELKGSETTFMCEYADETATIVEFLNRWITFSQSIISTLT

SEQ ID NO: 4 - protein, 132 aa, Artificial Sequence
  IL-2 analog 3
PTSSSTKKTQLQLEHLLLDLQMILNGINNYCNPKLTRMLTFKFYMPKKATELKHLQCLEEELKPLEEVLNLAQSKNFHLRPRDLISNINVIVLELKGSETTFMCEYADETATIVEFLNRWITFSQSIISTLT

SEQ ID NO: 5 - protein, 132 aa, Artificial Sequence
  IL-2 analog 4
PTSSSTKKTQLQLEHLLLDLQMILNGINNYKNPCLTRMLTFKFYMPKKATELKHLQCLEEELKPLEEVLNLAQSKNFHLRPRDLISNINVIVLELKGSETTFMCEYADETATIVEFLNRWITFSQSIISTLT

SEQ ID NO: 6 - protein, 132 aa, Artificial Sequence
  IL-2 analog 5
PTSSSTKKTQLQLEHLLLDLQMILNGINNYKNPKLTRMLTFCFYMPKKATELKHLQCLEEELKPLEEVLNLAQSKNFHLRPRDLISNINVIVLELKGSETTFMCEYADETATIVEFLNRWITFSQSIISTLT

SEQ ID NO: 7 - protein, 132 aa, Artificial Sequence
  IL-2 analog 6
PTSSSTKKTQLQLEHLLLDLQMILNGINNYKNPKLTRMLTFKFYMPCKATELKHLQCLEEELKPLEEVLNLAQSKNFHLRPRDLISNINVIVLELKGSETTFMCEYADETATIVEFLNRWITFSQSIISTLT

SEQ ID NO: 8 - protein, 132 aa, Artificial Sequence
  IL-2 analog 7
PTSSSTKKTQLQLEHLLLDLQMILNGINNYKNPKLTRMLTFKFYMPKCATELKHLQCLEEELKPLEEVLNLAQSKNFHLRPRDLISNINVIVLELKGSETTFMCEYADETATIVEFLNRWITFSQSIISTLT

SEQ ID NO: 9 - protein, 132 aa, Artificial Sequence
  IL-2 analog 9
PTSSSTKKTQLQLEHLLLDLQMILNGINNYKNPKLTRMLTFKFYMPKKATELKHLQCLEEELKPLEEVLNLAQSCNFHLRPRDLISNINVIVLELKGSETTFMCEYADETATIVEFLNRWITFSQSIISTLT

SEQ ID NO: 10 - protein, 132 aa, Artificial Sequence
  IL-2 analog 10
PTSSSTKKTQLQLEHLLLDLQMILNGINNYKNPKLTAMLTFKFYMPKKATELKHLQCLEEELKPLEEVLNLAQSKNFHLRPRDLISNINVIVLELKGSETTFMCEYADETATIVEFLNRWITFSQSIISTLT

SEQ ID NO: 11 - protein, 132 aa, Artificial Sequence
  IL-2 analog 10
PTSSSTKKTQLQLEHLLLDLQMILNGINNYKNPKLTRMLTKKFYMPKKATELKHLQCLEEELKPLEEVLNLAQSKNFHLRPRDLISNINVIVLELKGSETTFMCEYADETATIVEFLNRWITFSQSIISTLT

SEQ ID NO: 12 - protein, 132 aa, Artificial Sequence
  IL-2 analog 11
PTSSSTKKTQLQLEHLLLDLQMILNGINNYKNPKLTRMLTAKFYMPKKATELKHLQCLEEELKPLEEVLNLAQSKNFHLRPRDLISNINVIVLELKGSETTFMCEYADETATIVEFLNRWITFSQSIISTLT

SEQ ID NO: 13 - protein, 132 aa, Artificial Sequence
  IL-2 analog 12
PTSSSTKKTQLQLEHLLLDLQMILNGINNYKNPKLTAMLTKKFYMPKKATELKHLQCLEEELKPLEEVLNLAQSKNFHLRPRDLISNINVIVLELKGSETTFMCEYADETATIVEFLNRWITFSQSIISTLT

SEQ ID NO: 14 - protein, 132 aa, Artificial Sequence
  IL-2 analog 13
PTSSSTKKTQLQLEHLLLDLQMILNGINNYKNPKLTAMLTAKFYMPKKATELKHLQCLEEELKPLEEVLNLAQSKNFHLRPRDLISNINVIVLELKGSETTFMCEYADETATIVEFLNRWITFSQSIISTLT

SEQ ID NO: 15 - protein, 132 aa, Artificial Sequence
  IL-2 analog 14
PTSSSTKKTQLQLEHLLYDLQMILNGINNYKNPKLTAMLTKKFYMPKKATELKHLQCLEEELKPLEEVLNLAQSKNFHLRPRDLISNINVIVLELKGSETTFMCEYADETATIVEFLNRWITFSQSIISTLT

SEQ ID NO: 16 - protein, 132 aa, Artificial Sequence
  IL-2 analog 15
PTSSSTKKTQLQLEHLLLDLQMILNGINNYKNPKLTAMLTKKFYMPKKATELKHLQCLEEELKPLEEVLNLAQSKNFHLRPRELISNINVIVLELKGSETTFMCEYADETATIVEFLNRWITFSQSIISTLT

SEQ ID NO: 17 - protein, 132 aa, Artificial Sequence
  IL-2 analog 16
PTSSSTKKTQLQLEHLLLDLQMILNGINNYKNPKLTAMLTKKFYMPKKATELKHLQCLEEELKPLEEVLNLAQSKNFHLRPRDLISQINVIVLELKGSETTFMCEYADETATIVEFLNRWITFSQSIISTLT

SEQ ID NO: 18 - protein, 132 aa, Artificial Sequence
  IL-2 analog 17
PTSSSTKKTQLQLEHLLLDLQMILNGINNYKNPKLTAMLTKKFYMPKKATELKHLQCLEEELKPLEEVLNLAQSKNFHLRPRDLISNINTIVLELKGSETTFMCEYADETATIVEFLNRWITFSQSIISTLT

SEQ ID NO: 19 - protein, 132 aa, Artificial Sequence
  IL-2 analog 18
PTSSSTKKTQLQLEHLLLDLQMILNGINNYKNPKLTAMLTKKFYMPKKATELKHLQCLEQELKPLEEVLNLAQSKNFHLRPRDLISNINVIVLELKGSETTFMCEYADETATIVEFLNRWITFSQSIISTLT

SEQ ID NO: 20 - protein, 132 aa, Artificial Sequence
  IL-2 analog 19
PTSSSTKKTQLQLEHLLLDLQMILNGINNYKNPKLTAMLTKKFYMPKKATELKHLQCLEEELKPLEEVLNLAQSKNFHLDPRDLISNINVFVLELKGSETTFMCEYADETATIVEFLNRWITFSQSIISTLT

SEQ ID NO: 21 - protein, 132 aa, Artificial Sequence
  IL-2 analog 20
PTSSSTKKTQLQLEHLLLDLQMILNGINNYKNPKLTAMLTKKFYMPKKATELKHLQCLEEELKPLEEVLNLAQSKNFHLRPRDVVSNINVFVLELKGSETTFMCEYADETATIVEFLNRWITFSQSIISTLT

SEQ ID NO: 22 - protein, 132 aa, Artificial Sequence
  IL-2 analog 21
PTSSSTKKTQLQLEHLLLDLQMILNGINNYKNPKLTAMLTKKFYMPKKATELKHLQCLEEELKPLEEVLNLAQSKNFHFDPRDVVSNINVFVLELKGSETTFMCEYADETATIVEFLNRWITFSQSIISTLT

SEQ ID NO: 23 - protein, 132 aa, Artificial Sequence
  IL-2 analog 22
PTSSSTKKTQVQLEHLLLDLQMILNGINNYKNPKLTAMLTKKFYMPKKATELKHLQCLEEELKPLEEVLNLAQSKNFHLRPRDLISNINVIVLELKGSETTFMCEYADETATIVEFLNRWITFSQSIISTLT

SEQ ID NO: 24 - protein, 132 aa, Artificial Sequence
  IL-2 analog 23
PTSSSTKKTQFQLEHLLLDLQMILNGINNYKNPKLTAMLTKKFYMPKKATELKHLQCLEEELKPLEEVLNLAQSKNFHLRPRDLISNINVIVLELKGSETTFMCEYADETATIVEFLNRWITFSQSIISTLT

SEQ ID NO: 25 - protein, 132 aa, Artificial Sequence
  IL-2 analog 24
PTSSSTKKTQLQLEHLLVDLQMILNGINNYKNPKLTAMLTKKFYMPKKATELKHLQCLEEELKPLEEVLNLAQSKNFHLRPRDLISNINVIVLELKGSETTFMCEYADETATIVEFLNRWITFSQSIISTLT

SEQ ID NO: 26 - protein, 132 aa, Artificial Sequence
  IL-2 analog 25
PTSSSTKKTQLQLEHLLFDLQMILNGINNYKNPKLTAMLTKKFYMPKKATELKHLQCLEEELKPLEEVLNLAQSKNFHLRPRDLISNINVIVLELKGSETTFMCEYADETATIVEFLNRWITFSQSIISTLT

SEQ ID NO: 27 - protein, 132 aa, Artificial Sequence
  IL-2 analog 26
PTSSSTKKTQLQLEHLLLDLQMILNGINNYKNPKLTAMLTKKFYMPKKATELKHLQCLEEELKPLEEVLNLAQSKNFHLRPRDLISNFNVIVLELKGSETTFMCEYADETATIVEFLNRWITFSQSIISTLT

SEQ ID NO: 28 - protein, 132 aa, Artificial Sequence
  IL-2 analog 27
PTSSSTKKTQLQLEHLLLDLQMILNGINNYKNPKLTAMLTKKFYMPKKATELKHLQCLEEELKPLEEVLNLAQSKNFHLRPRDLISNINFIVLELKGSETTFMCEYADETATIVEFLNRWITFSQSIISTLT

SEQ ID NO: 29 - protein, 132 aa, Artificial Sequence
  IL-2 analog 28
PTSSSTKKTQLQLEHLLLDLQMILNGINNYKNPKLTAMLTKKFYMPKKATELKHLQCLEEELKPLEEVLNLAQSKNFHLRPRDLISNINVIVVELKGSETTFMCEYADETATIVEFLNRWITFSQSIISTLT

SEQ ID NO: 30 - protein, 132 aa, Artificial Sequence
  IL-2 analog 29
PTSSSTKKTQLQLEHLLLDLQMILNGINNYKNPKLTAMLTKKFYMPKKATELKHLQCLEEELKPLEEVLNLAQSKNFHLRPRDLISNINVIVLELKGSETTFMCEYADETATIVEFLNRWITFSTSIISTLT

SEQ ID NO: 31 - protein, 132 aa, Artificial Sequence
  IL-2 analog 30
PTSSSTKKTQLQLEHLLLDLQMILNGINNYKNPKLTAMLTFKFYMPKKATELKHLQCLEEELKPLEEVLNLAQSKNFHLDPRDLISNINVFVLELKGSETTFMCEYADETATIVEFLNRWITFSQSIISTLT

SEQ ID NO: 32 - protein, 132 aa, Artificial Sequence
  IL-2 analog 31
PTSSSTKKTQLQLEHLLLDLQMILNGINNYKNPKLTAMLTFKFYMPKKATELKHLQCLEEELKPLEEVLNLAQSKNFHLRPRELISNINVIVLELKGSETTFMCEYADETATIVEFLNRWITFSQSIISTLT

SEQ ID NO: 33 - protein, 132 aa, Artificial Sequence
  IL-2 analog 32
PTSSSTKKTQLQLEHLLLDLQMILNGINNYKNPKLTAMLTFKFYMPKKATELKHLQCLEEELKPLEEVLNLAQSKNFHLDPRELISNINVFVLELKGSETTFMCEYADETATIVEFLNRWITFSQSIISTLT

SEQ ID NO: 34 - protein, 132 aa, Artificial Sequence
  IL-2 analog 33
PTSSSTKKTQLQLEHLLLDLQMILNGINNYKNPKLTAMLTFKFYMPKKATELKHLQCLEEELKPLEEVLNLAQSKNFHFRPRDLISNINVIVLELKGSETTFMCEYADETATIVEFLNRWITFSQSIISTLT

SEQ ID NO: 35 - protein, 132 aa, Artificial Sequence
  IL-2 analog 34
PTSSSTKKTQLQLEHLLLDLQMILNGINNYKNPKLTAMLTFKFYMPKKATELKHLQCLEEELKPLEEVLNLAQSKNFHFRPRELISNINVIVLELKGSETTFMCEYADETATIVEFLNRWITFSQSIISTLT

SEQ ID NO: 36 - protein, 132 aa, Artificial Sequence
  IL-2 analog 35
PTSSSTKKTQLQLEHLLLDLQMILNGINNYKNPKLTAMLTFKFYMPKKATELKHLQCLEEELKPLEEVLNLAQSKNFHLRPRDLISNINVIVFEFKGSETTFMCEYADETATIVEFLNRWITFSQSIISTLT

SEQ ID NO: 37 - protein, 132 aa, Artificial Sequence
  IL-2 analog 36
PTSSSTKKTQLQLEHLLLDLQMILNGINNYKNPKLTAMLTFKFYMPKKATELKHLQCLEEELKPLEEVLNLAQSKNFHLRPRDLISNINVIVFEVKGSETTFMCEYADETATIVEFLNRWITFSQSIISTLT

SEQ ID NO: 38 - protein, 132 aa, Artificial Sequence
  IL-2 analog 37
PTSSSTKKTQLQLEHLLLDLQMILNGINNYKNPKLTAMLTFKFYMPKKATELKHLQCLEEELKPLEEVLNLAQSKNFHLRPRDLISNINVIVFEIKGSETTFMCEYADETATIVEFLNRWITFSQSIISTLT

SEQ ID NO: 39 - protein, 132 aa, Artificial Sequence
  IL-2 analog 38
PTSSSTKKTQLQLEHLLLDLQMILNGINNYKNPKLTAMLTFKFYMPKKATELKHLQCLEEELKPLEEVLNLAQSKNFHLDPRDLISNINVFVFEFKGSETTFMCEYADETATIVEFLNRWITFSQSIISTLT

SEQ ID NO: 40 - protein, 132 aa, Artificial Sequence
  IL-2 analog 39
PTSSSTKKTQLQLEHLLLDLQMILNGINNYKNPKLTAMLTFKFYMPKKATELKHLQCLEEELKPLEEVLNLAQSKNFHLDPRDLISNINVFVFEVKGSETTFMCEYADETATIVEFLNRWITFSQSIISTLT

SEQ ID NO: 41 - protein, 132 aa, Artificial Sequence
  IL-2 analog 40
PTSSSTKKTQLQLEHLLLDLQMILNGINNYKNPKLTAMLTKKFYMPKKATELKHLQCLEEELKPLEEVLNLAQSKNFHLDPRDLISNINVFVFEIKGSETTFMCEYADETATIVEFLNRWITFSQSIISTLT

SEQ ID NO: 42 - protein, 132 aa, Artificial Sequence
  IL-2 analog 41
PTSSSTKKTQLQLEHLLLDLQMILNGINNYKNPKLTRMLTFKFYMPKKATELKHLQCLEEELKPLEEVLNLAQSKNFHFDPRDVVSNINVFVLELKGSETTFMCEYADETATIVEFLNRWITFSQSIISTLT

SEQ ID NO: 43 - protein, 132 aa, Artificial Sequence
  IL-2 analog 42
PTSSSTKKTQLQLEHLLLDLQMILNGINNYKNPKLTAMLTKKFYMPKKATELKHLQCLEEELKPLEEVLNLAQSKNFHLEPRDLISNINVFVLELKGSETTFMCEYADETATIVEFLNRWITFSQSIISTLT

SEQ ID NO: 44 - protein, 132 aa, Artificial Sequence
  IL-2 analog 43
PTSSSTKKTQLQLEHLLLDLQMILNGINNYKNPKLTAMLTKKFYMPKKATELKHLQCLEEELKPLEEVLNLAQSKNFHLDPRDLISNINVLVLELKGSETTFMCEYADETATIVEFLNRWITFSQSIISTLT

SEQ ID NO: 45 - protein, 132 aa, Artificial Sequence
  IL-2 analog 44
PTSSSTKKTQLQLEHLLLDLQMILNGINNYKNPKLTAMLTKKFYMPKKATELKHLQCLEEELKPLEEVLNLAQSKNFHLDPRVLISNINVFVLELKGSETTFMCEYADETATIVEFLNRWITFSQSIISTLT

SEQ ID NO: 46 - protein, 132 aa, Artificial Sequence
  IL-2 analog 45
PTSSSTKKTQLQLEHLLLDLQMILNGINNYKNPKLTAMLTKKFYMPKKATELKHLQCLEEELKPLEEVLNLAQSKNFHLDPRFLISNINVFVLELKGSETTFMCEYADETATIVEFLNRWITFSQSIISTLT

SEQ ID NO: 47 - protein, 132 aa, Artificial Sequence
  IL-2 analog 46
PTSSSTKKTQLQLEHLLLVLQMILNGINNYKNPKLTAMLTKKFYMPKKATELKHLQCLEEELKPLEEVLNLAQSKNFHLDPRDLISNINVFVLELKGSETTFMCEYADETATIVEFLNRWITFSQSIISTLT

SEQ ID NO: 48 - protein, 132 aa, Artificial Sequence
  IL-2 analog 47
PTSSSTKKTQLQLEHLLLFLQMILNGINNYKNPKLTAMLTKKFYMPKKATELKHLQCLEEELKPLEEVLNLAQSKNFHLDPRDLISNINVFVLELKGSETTFMCEYADETATIVEFLNRWITFSQSIISTLT

SEQ ID NO: 49 - protein, 132 aa, Artificial Sequence
  IL-2 analog 48
PTSSSTKKTQLQLEHLLLDLQMILNGINNYKNPKLTAMLTKKFYMPKKATELKHLQCLEEELKPLEEVLNLAQSKNFHLDPRDLISVINVFVLELKGSETTFMCEYADETATIVEFLNRWITFSQSIISTLT

SEQ ID NO: 50 - protein, 132 aa, Artificial Sequence
  IL-2 analog 49
PTSSSTKKTQLQLEHLLLDLQMILNGINNYKNPKLTAMLTKKFYMPKKATELKHLQCLEEELKPLEEVLNLAQSKNFHLDPRDLISFINVFVLELKGSETTFMCEYADETATIVEFLNRWITFSQSIISTLT

SEQ ID NO: 51 - protein, 132 aa, Artificial Sequence
  IL-2 analog 50
PTSSSTKKTQLQLEHLLLDLQMILNGINNYKNPKLTRMLTKKFYMPKKATELKHLQCLEEELKPLEEVLNLAQSKNFHFDPRDVVSNINVFVLELKGSETTFMCEYADETATIVEFLNRWITFSQSIISTLT

SEQ ID NO: 52 - protein, 132 aa, Artificial Sequence
  IL-2 analog 51
PTSSSTKKTQLQLEHLLLDLQMILNGINNYKNPKLTRMLTFKFYMPKKATELKHLQCLEQELKPLEEVLNLAQSKNFHLDPRDLISNINVFVLELKGSETTFMCEYADETATIVEFLNRWITFSQSIISTLT

SEQ ID NO: 53 - protein, 132 aa, Artificial Sequence
  IL-2 analog 52
PTSSSTKKTQLQLEHLLLDLQMILNGINNYKNPKLTAMLTKKFYMPKKATELKHLQCLEEELKPLEEVLNLAQSKNFHFDPRDLISNINVFVLELKGSETTFMCEYADETATIVEFLNRWITFSQSIISTLT

SEQ ID NO: 54 - protein, 132 aa, Artificial Sequence
  IL-2 analog 53
PTSSSTKKTQLQLEHLLLDLQMILNGINNYKNPKLTAMLTKKFYMPKKATELKHLQCLEEELKPLEEVLNLAQSKNFHFDPRELISNINVFVLELKGSETTFMCEYADETATIVEFLNRWITFSQSIISTLT

SEQ ID NO: 55 - protein, 132 aa, Artificial Sequence
  IL-2 analog 54
PTSSSTKKTQLQLEHLLLDLQMILNGINNYKNPKLTAMLTKKFYMPKKATELKHLQCLEEELKPLEEVLNLAHSKNFHLDPRDLISNINVFVLELKGSETTFMCEYADETATIVEFLNRWITFSQSIISTLT

SEQ ID NO: 56 - protein, 132 aa, Artificial Sequence
  IL-2 analog 55
PTSSSTKKTQLQLEHLLLDLQMILNGINNYKNPKLTAMLTKKFYMPKKATELKHLQCLEEELKPLEEVLNLAHSKNFHFDPRDLISNINVFVLELKGSETTFMCEYADETATIVEFLNRWITFSQSIISTLT

SEQ ID NO: 57 - protein, 132 aa, Artificial Sequence
  IL-2 analog 56
PTSSSTKKTQLQLEHLLLDLQMILNGINNYKNPKLTAMLTKKFAMPKKATELKHLQCLEEELKPLEEVLNLAHSKNFHLDPRDLISNINVFVLELKGSETTFMCEYADETATIVEFLNRWITFSQSIISTLT

SEQ ID NO: 58 - protein, 132 aa, Artificial Sequence
  IL-2 analog 57
PTSSSTKKTQLQLEHLLLDLQMILNGINNYKNPKLTAMLTKKFAMPKKATELKHLQCLEEELKPLEEVLNLAHSKNFHFDPRDLISNINVFVLELKGSETTFMCEYADETATIVEFLNRWITFSQSIISTLT

SEQ ID NO: 59 - protein, 132 aa, Artificial Sequence
  IL-2 analog 61
PTSSSTKKTQLQLEHLLLDLQMILNGINNYKNPKLTAMLTKKFYMPKKATELKHLQCLEEELKPLEEVLNLAQSKNFHYDPRDGVSNINVYVLELKGSETTFMCEYADETATIVEFLNRWITFSQSIISTLT

SEQ ID NO: 60 - protein, 132 aa, Artificial Sequence
  IL-2 analog 59
PTSSSTKKTQLQLEHLLLDLQMILNGINNYKNPKLTAMLTKKFYMPKKATELKHLQCLEEELKPLEEVLNLAQSKNFHFDPRDAASNINVYVLELKGSETTFMCEYADETATIVEFLNRWITFSQSIISTLT

SEQ ID NO: 61 - protein, 132 aa, Artificial Sequence
  IL-2 analog 60
PTSSSTKKTQLQLEHLLLDLQMILNGINNYKNPKLTAMLTKKFAMPKKATELKHLQCLEEELKPLEEVLNLAQSKNFHYRPRDAASNINVYVLELKGSETTFMCEYADETATIVEFLNRWITFSQSIISTLT

SEQ ID NO: 62 - protein, 132 aa, Artificial Sequence; identical to SEQ ID NO: 59
  IL-2 analog 61

SEQ ID NO: 63 - protein, 132 aa, Artificial Sequence
  IL-2 analog 62
PTSSSTKKTQLQLEHLLLDLQMILNGINNYKNPKLTAMLTKKFYMPKKATELKHLQCLEEELKPLEEVLNLAQSKNFHWEPRDGASNINVFVLELKGSETTFMCEYADETATIVEFLNRWITFSQSIISTLT

SEQ ID NO: 64 - protein, 132 aa, Artificial Sequence
  IL-2 analog 63
PTSSSTKKTQLQLEHLLLDLQMILNGINNYKNPKLTAMLTKKFYMPKKATELKHLQCLEEELKPLEEVLNLAQSKNFHDEPRDTGSNINVFVLELKGSETTFMCEYADETATIVEFLNRWITFSQSIISTLT

SEQ ID NO: 65 - protein, 132 aa, Artificial Sequence
  IL-2 analog 64
PTSSSTKKTQLQLEHLLLDLQMILNGINNYKNPKLTAMLTKKFYMPKKATELKHLQCLEEELKPLEEVLNLAQSKNFHYNPRDVVSNINVYVLELKGSETTFMCEYADETATIVEFLNRWITFSQSIISTLT

SEQ ID NO: 66 - protein, 132 aa, Artificial Sequence
  IL-2 analog 65
PTSSSTKKTQLQLEHLLLDLQMILNGINNYKNPKLTAMLTKKFYMPKKATELKHLQCLEEELKPLEEVLNLAQSKNFHYEPRDVVSNINVFVLELKGSETTFMCEYADETATIVEFLNRWITFSQSIISTLT

SEQ ID NO: 67 - protein, 132 aa, Artificial Sequence
  IL-2 analog 66
PTSSSTKKTQLQLEHLLLDLQMILNGINNYKNPKLTAMLTKKFYMPKKATELKHLQCLEEELKPLEEVLNLAQSKNFHFEPRDFVSNINVFVLELKGSETTFMCEYADETATIVEFLNRWITFSQSIISTLT

SEQ ID NO: 68 - protein, 132 aa, Artificial Sequence
  IL-2 analog 67
PTSSSTKKTQLQLEHLLLDLQMILNGINNYKNPKLTAMLTKKFYMPKKATELKHLQCLEEELKPLEEVLNLAQSKNFHYDPRDFVSNINVWVLDLKGSETTFMCEYADETATIVEFLNRWITFSQSIISTLT

SEQ ID NO: 69 - protein, 132 aa, Artificial Sequence
  IL-2 analog 68
PTSSSTKKTQLQLEHLLLDLQMILNGINNYKNPKLTAMLTKKFYMPKKATELKHLQCLEEELKPLEEVLNLAQSKNFHFEPRDIVSNINEFVLELKGSETTFMCEYADETATIVEFLNRWITFSQSIISTLT

SEQ ID NO: 70 - protein, 132 aa, Artificial Sequence
  IL-2 analog 69
PTSSSTKKTQLQLEHLLLDLQMILNGINNYKNPKLTAMLTKKFYMPKKATELKHLQCLEEELKPLEEVLNLAQSKNFHYEPRDFLSNINEWVLDLKGSETTFMCEYADETATIVEFLNRWITFSQSIISTLT

SEQ ID NO: 71 - protein, 132 aa, Artificial Sequence
  IL-2 analog 70
PTSSSTKKTQLQLEHLLLDLQMILNGINNYKNPKLTAMLTKKFYMPKKATELKHLQCLEEELKPLEEVLNLAQSKNFHYDPRDVVSNINVFVLELKGSETTFMCEYADETATIVEFLNRWITFSQSIISTLT

SEQ ID NO: 72 - protein, 132 aa, Artificial Sequence
  IL-2 analog 71
PTSSSTKKTQLQLEHLLLDLQMILNGINNYKNPKLTAMLTKKFYMPKKATELKHLQCLEEELKPLEEVLNLAQSKNFHFEPRDVVSNINVFVLELKGSETTFMCEYADETATIVEFLNRWITFSQSIISTLT

SEQ ID NO: 73 - protein, 132 aa, Artificial Sequence
  IL-2 analog 72
PTSSSTKKTQLQLEHLLLDLQMILNGINNYKNPKLTAMLTKKFYMPKKATELKHLQCLEEELKPLEEVLNLAQSKNFHFDPRDVGSNINVFVLELKGSETTFMCEYADETATIVEFLNRWITFSQSIISTLT

SEQ ID NO: 74 - protein, 132 aa, Artificial Sequence
  IL-2 analog 73
PTSSSTKKTQLQLEHLLLDLQMILNGINNYKNPKLTAMLTKKFYMPKKATELKHLQCLEEELKPLEEVLNLAQSKNFHFDPRDWVSNINVFVLELKGSETTFMCEYADETATIVEFLNRWITFSQSIISTLT

SEQ ID NO: 75 - protein, 132 aa, Artificial Sequence
  IL-2 analog 74
PTSSSTKKTQLQLEHLLLDLQMILNGINNYKNPKLTDMLTKKFYMPKKATELKHLQCLEEELKPLEEVLNLAQSKNFHYDPRDVVSNINVFVLELKGSETTFMCEYADETATIVEFLNRWITFSQSIISTLT

SEQ ID NO: 76 - protein, 132 aa, Artificial Sequence
  IL-2 analog 75
PTSSSTKKTQLQLEHLLLDLQMILNGINNYKNPKLTAMLTKKFAMPKKATELKHLQCLEEELKPLEEVLNLAQSKNFHFEPRDVVSNINVFVLELKGSETTFMCEYADETATIVEFLNRWITFSQSIISTLT

SEQ ID NO: 77 - protein, 132 aa, Artificial Sequence
  IL-2 analog 76
PTSSSTKKTQLQLEHLLLDLQMILNGINNYKNPKLTAMLTKQFYMPKKATELKHLQCLERELKPLEEVLNLAQSKNFHFDPRDVGSNINVFVLELKGSETTFMCEYADETATIVEFLNRWITFSQSIISTLT

SEQ ID NO: 78 - protein, 132 aa, Artificial Sequence
  IL-2 analog 77
PTSSSTKKTQLQLEHLLLDLQMILNGINNYKNPKLTAMLTKEFYMPKKATELKHLQCLERELKPLEEVLNLAQSKNFHFDPRDWVSNINVFVLELKGSETTFMCEYADETATIVEFLNRWITFSQSIISTLT

SEQ ID NO: 79 - protein, 132 aa, Artificial Sequence
  IL-2 analog 78
PTSSSTKKTQLQLEHLLLDLQMILNGINNYKNPELTAMLTKKFYMPKKATELKHLQCLEEELKPLEEVLNLAQSKNFHFEPRDVVSNINVFVLELKGSETTFMCEYADETATIVEFLNRWITFSQSIISTLT

SEQ ID NO: 80 - protein, 132 aa, Artificial Sequence
  IL-2 analog 79
PTSSSTKKTQLQLEHLLLDLQMILNGINNYKNPELTAMLTKKFYMPKKATELKHLQCLEEELKPLEEVLNLAHSKNFHFEPRDVVSNINVFVLELKGSETTFMCEYADETATIVEFLNRWITFSQSIISTLT

SEQ ID NO: 81 - protein, 132 aa, Artificial Sequence
  IL-2 analog 80
PTSSSTKKTQLQLEHLLLDLQMILNGINNYKNPELTAMLTKKFYMPKKATELKHLQCLEEELKPLEEVLNLAHSKNFHFEGRDVVSNINVFVLELKGSETTFMCEYADETATIVEFLNRWITFSQSIISTLT

SEQ ID NO: 82 - protein, 132 aa, Artificial Sequence
  IL-2 analog 81
PTSSSTKKTQLQLEHLLLDLQMILNGINNYKNPELTAMLTKKFYMPKKATELKHLQCLEEELKPLEEVLNLAHSKNFHFEVRDVVSNINVFVLELKGSETTFMCEYADETATIVEFLNRWITFSQSIISTLT

SEQ ID NO: 83 - protein, 132 aa, Artificial Sequence
  IL-2 analog 82
PTSSSTKKTQLQLEHLRLDLEMILNGINNYKNPKLTRMLTFKFYMPKKATELKHLQCLEEELKPLEEVLNLAQSKNFHFDPRDEVSNINVFVLELKGSETTFMCEYADETATIVEFLNRWITFSQSIISTLT

SEQ ID NO: 84 - protein, 132 aa, Artificial Sequence
  IL-2 analog 83
PTSSSTKKTQLQLEHLRRDLEMILNGINNYKNPKLTRMLTFKFYMPKKATELKHLQCLEEELKPLEEVLNLAQSKNFHFDPRDEVSNINVFVLELKGSETTFMCEYADETATIVEFLNRWITFSQSIISTLT

SEQ ID NO: 85 - protein, 132 aa, Artificial Sequence
  IL-2 analog 84
PTSSSTKKTQLQLEHLRLDLEMILNGINNYKNPKLTRMLTFKFYMPKKATELKHLQCLEEELKPLEEVLNLAQSKNFHVDPRDEVSNINVFVLELKGSETTFMCEYADETATIVEFLNRWITFSQSIISTLT

SEQ ID NO: 86 - protein, 132 aa, Artificial Sequence
  IL-2 analog 85
PTSSSTKKTQLQLEHLLLDLQMILNGINNYKNPKLTRMLTFKFYMPKKATELKHLQCLEEELKPLEEVLNLAQSKNFHFEPRDVVSNINVFVLELKGSETTFMCEYADETATIVEFLNRWITFSQSIISTLT

SEQ ID NO: 87 - protein, 132 aa, Artificial Sequence
  IL-2 analog 86
PTSSSTKKTQLQLEHLRLDLEMILNGINNYKNPKLTRMLTFKFYMPKKATELKHLQCLEEELKPLEEVLNLAQSKNFHFEPRDVVSNINVFVLELKGSETTFMCEYADETATIVEFLNRWITFSQSIISTLT

SEQ ID NO: 88 - protein, 132 aa, Artificial Sequence
  IL-2 analog 87
PTSSSTKKTQLQLEHLRRDLEMILNGINNYKNPKLTRMLTFKFYMPKKATELKHLQCLEEELKPLEEVLNLAQSKNFHFEPRDVVSNINVFVLELKGSETTFMCEYADETATIVEFLNRWITFSQSIISTLT

SEQ ID NO: 89 - protein, 132 aa, Artificial Sequence
  IL-2 analog 88
PTSSSTKKTQLQLEHLLLDLQMILNGINNYKNPKLTRMLTFKFYMPKKATELKHLQCLEDELKPLEEVLNLAQSKNFHFEPRDVVSNINVFVLELKGSETTFMCEYADETATIVEFLNRWITFSQSIISTLT

SEQ ID NO: 90 - protein, 132 aa, Artificial Sequence
  IL-2 analog 89
PTSSSTKKTQLQLEHLLLDLQMILNGINNYKNPKLTAMLTFKFYMPKKATELKHLQCLEEELKPLEQVLNLAQSKNFHFEPRDVVSNINVFVLELKGSETTFMCEYADETATIVEFLNRWITFSQSIISTLT

SEQ ID NO: 91 - protein, 132 aa, Artificial Sequence
  IL-2 analog 90
PTSSSTKKTQLQLEHLLLDLQMILNGINNYKNPKLTRMLTWKFYMPKKATELKHLQCLEEELKPLEEVLNLAQSKNFHFEPRDVVSNINVFVLELKGSETTFMCEYADETATIVEFLNRWITFSQSIISTLT

SEQ ID NO: 92 - protein, 132 aa, Artificial Sequence
  IL-2 analog 91
PTSSSTKKTQLQLEHLLLDLQMILNGINNYKNPKLTRMLTFKFYMPKKATELKHLQCLEQELKPLEEVLNLAQSKNFHFEPRDVVSNINVFVLELKGSETTFMCEYADETATIVEFLNRWITFSQSIISTLT

SEQ ID NO: 93 - protein, 132 aa, Artificial Sequence
  IL-2 analog 92
PTSSSTKKTQLQLEHLLLDLQMILNGINNYKNPKLTRMLTFKFYMPKKATELKHLQCLEEELKPLEEVLNLAQSKNFHFEPRDVVSNINTFVLELKGSETTFMCEYADETATIVEFLNRWITFSQSIISTLT

SEQ ID NO: 94 - protein, 132 aa, Artificial Sequence
  IL-2 analog 93
PTSSSTKKTQLQLEHLLLDLQMILNGINNYKNPKLTRMLTFKFYMPKKATELKHLQCLEEELKPLEEVLNLAQSKNFHFEPREVVSNINTFVLELKGSETTFMCEYADETATIVEFLNRWITFSQSIISTLT

SEQ ID NO: 95 - protein, 132 aa, Artificial Sequence
  IL-2 analog 94
PTSSSTKKTQLQLEHLLLDLQMILNGINNYKNPKLTRMLTFKFYMPKKATELKHLQCLEEELKPLEEVLNLAQSKNFHFEPRDVVSNINVFVFEFKGSETTFMCEYADETATIVEFLNRWITFSQSIISTLT

SEQ ID NO: 96 - protein, 132 aa, Artificial Sequence
  IL-2 analog 95
PTSSSTKKTQLQLEHLLLDLQMILNGINNYKNPKLTRMLTFKFYMPKKATELKHLQCLEEELKPLEEGLNLAQSKNFHFEPRDVVSNINVFVLELKGSETTFMCEYADETATIVEFLNRWITFSQSIISTLT

SEQ ID NO: 97 - protein, 132 aa, Artificial Sequence
  IL-2 analog 96
PTSSSTKKTQLQLEHLLLDLQMILNGINNYKNPKLTRMLTFKFYMPKKATELKHLQCLEEELKPLEEGLNLAASKNFHFEPRDVVSNINVFVLELKGSETTFMCEYADETATIVEFLNRWITFSQSIISTLT

SEQ ID NO: 98 - protein, 132 aa, Artificial Sequence
  IL-2 analog 97
PTSSSTKKTQLQLEHLLLDLQMILNGINNYKNPKLTAMLTFKFYMPKKATELKHLQCLEEELKPLEEVLNLAQSKNFHFDPRDLISNINVFVLELKGSETTFMCEYADETATIVEFLNRWITFSQSIISTLT

SEQ ID NO: 99 - protein, 132 aa, Artificial Sequence
  IL-2 analog 98
PTSSSTKKTQLQLEHLLLDLQMILNGINNYKNPKLTAMLTFKFYMPKKATELKHLQCLEEELKPLEEVLNLAQSKNFHFEPRDVISNINVFVLELKGSETTFMCEYADETATIVEFLNRWITFSQSIISTLT

SEQ ID NO: 100 - protein, 132 aa, Artificial Sequence
  IL-2 analog 99
PTSSSTKKTQLQLEHLLLDLQMILNGINNYKNPKLTAMLTFKFYMPKKATELKHLQCLEEELKPLEEVLNLAQSKNFHFEPRDLVSNINVFVLELKGSETTFMCEYADETATIVEFLNRWITFSQSIISTLT

SEQ ID NO: 101 - protein, 132 aa, Artificial Sequence
  IL-2 analog 100
PTSSSTKKTQLQLEHLLLDLQMILNGINNYKNPKLTRMLTFKFYMPKKATELKHLQCLEEELKPLEEVLNLAQSKNFHFEPRDYVSNINVFVLELKGSETTFMCEYADETATIVEFLNRWITFSQSIISTLT

SEQ ID NO: 102 - protein, 132 aa, Artificial Sequence
  IL-2 analog 101
PTSSSTKKTQLQLEHLLLDLQMILNGINNYKNPKLTRMLTFKFYMPKKATELKHLQCLEEELKPLEEVLNLAQSKNFHFEPRDLASNINVFVLELKGSETTFMCEYADETATIVEFLNRWITFSQSIISTLT

SEQ ID NO: 103 - protein, 132 aa, Artificial Sequence
  IL-2 analog 102
PTSSSTKKTQLQLEHLLLDLQMILNGINNYKNPKLTRMLTFKFYMPKKATELKHLQCLEEELKPLEEVLNLAQSKNFHFEPRDVVSNINVIVLELKGSETTFMCEYADETATIVEFLNRWITFSQSIISTLT

SEQ ID NO: 104 - protein, 132 aa, Artificial Sequence
  IL-2 analog 103
PTSSSTKKTQLQLEHLRLDLEMILNGINNYKNPKLTAMLTFKFYMPKKATELKHLQCLEEELKPLEEVLNLAQSKNFHFEPRDVVSNINVFVLELKGSETTFMCEYADETATIVEFLNRWITFSQSIISTLT

SEQ ID NO: 105 - protein, 132 aa, Artificial Sequence
  IL-2 analog 104
PTSSSTKKTQLQLEHLRLDLEMILNGINNYKNPKLTRMLTFKFYMPKKATELKHLQCLEDELKPLEEVLNLAQSKNFHFEPRDVVSNINVFVLELKGSETTFMCEYADETATIVEFLNRWITFSQSIISTLT

SEQ ID NO: 106 - protein, 132 aa, Artificial Sequence
  IL-2 analog 105
PTSSSTKKTQLQLEHLRLDLEMILNGINNYKNPKLTRMLTFKFYMPKKATELKHLQCLEEELKPLEDVLNLAQSKNFHFEPRDVVSNINVFVLELKGSETTFMCEYADETATIVEFLNRWITFSQSIISTLT

SEQ ID NO: 107 - DNA, 399 bp, Artificial Sequence
  IL-2 analog 1
cctacttcaagttctacaaagaaaacacagctacaactggagcatttactgctggatttacagatgattttgaatggaattaataattacaagaatcccaaactcaccaggatgctcacatttaagttttacatgcccaagaaggccacagaactgaaacatcttcagtgtctagaagaagaactcaaacctctggaggaagtgctaaatttagctcaaagcaaaaactttcacttaagacccagggacttaatcagcaatatcaacgtaatagttctggaactaaagggatctgaaacaacattcatgtgtgaatatgctgatgagacagcaaccattgtagaatttctgaacagatggattacctttagtcaaagcatcatctcaacactgacttga

SEQ ID NO: 108 - DNA, 399 bp, Artificial Sequence
  IL-2 analog 2
cctacttcaagttctacaaagaaaacacagctacaactggagcatttactgctggatttacagatgattttgaatggaattaataattacaagaatcccaaactcaccaggatgctcacatttaagttttacatgcccaagaaggccacagaactgaaacatcttcagtgtctagaagaagaactcaaacctctggaggaagtgctaaatttagctcaaagcaaaaactttcacttaagacccagggacttaatctgcaatatcaacgtaatagttctggaactaaagggatctgaaacaacattcatgtgtgaatatgctgatgagacagcaaccattgtagaatttctgaacagatggattacctttagtcaaagcatcatctcaacactgacttga

SEQ ID NO: 109 - DNA, 399 bp, Artificial Sequence
  IL-2 analog 3
cctacttcaagttctacaaagaaaacacagctacaactggagcatttactgctggatttacagatgattttgaatggaattaataattactgtaatcccaaactcaccaggatgctcacatttaagttttacatgcccaagaaggccacagaactgaaacatcttcagtgtctagaagaagaactcaaacctctggaggaagtgctaaatttagctcaaagcaaaaactttcacttaagacccagggacttaatcagcaatatcaacgtaatagttctggaactaaagggatctgaaacaacattcatgtgtgaatatgctgatgagacagcaaccattgtagaatttctgaacagatggattacctttagtcaaagcatcatctcaacactgacttga

SEQ ID NO: 110 - DNA, 399 bp, Artificial Sequence
  IL-2 analog 4
cctacttcaagttctacaaagaaaacacagctacaactggagcatttactgctggatttacagatgattttgaatggaattaataattacaagaatccctgtctcaccaggatgctcacatttaagttttacatgcccaagaaggccacagaactgaaacatcttcagtgtctagaagaagaactcaaacctctggaggaagtgctaaatttagctcaaagcaaaaactttcacttaagacccagggacttaatcagcaatatcaacgtaatagttctggaactaaagggatctgaaacaacattcatgtgtgaatatgctgatgagacagcaaccattgtagaatttctgaacagatggattacctttagtcaaagcatcatctcaacactgacttga

SEQ ID NO: 111 - DNA, 399 bp, Artificial Sequence
  IL-2 analog 5
cctacttcaagttctacaaagaaaacacagctacaactggagcatttactgctggatttacagatgattttgaatggaattaataattacaagaatcccaaactcaccaggatgctcacattttgtttttacatgcccaagaaggccacagaactgaaacatcttcagtgtctagaagaagaactcaaacctctggaggaagtgctaaatttagctcaaagcaaaaactttcacttaagacccagggacttaatcagcaatatcaacgtaatagttctggaactaaagggatctgaaacaacattcatgtgtgaatatgctgatgagacagcaaccattgtagaatttctgaacagatggattacctttagtcaaagcatcatctcaacactgacttga

SEQ ID NO: 112 - DNA, 399 bp, Artificial Sequence
  IL-2 analog 6
cctacttcaagttctacaaagaaaacacagctacaactggagcatttactgctggatttacagatgattttgaatggaattaataattacaagaatcccaaactcaccaggatgctcacatttaagttttacatgccctgtaaggccacagaactgaaacatcttcagtgtctagaagaagaactcaaacctctggaggaagtgctaaatttagctcaaagcaaaaactttcacttaagacccagggacttaatcagcaatatcaacgtaatagttctggaactaaagggatctgaaacaacattcatgtgtgaatatgctgatgagacagcaaccattgtagaatttctgaacagatggattacctttagtcaaagcatcatctcaacactgacttga

SEQ ID NO: 113 - DNA, 399 bp, Artificial Sequence
  IL-2 analog 7
cctacttcaagttctacaaagaaaacacagctacaactggagcatttactgctggatttacagatgattttgaatggaattaataattacaagaatcccaaactcaccaggatgctcacatttaagttttacatgcccaagtgtgccacagaactgaaacatcttcagtgtctagaagaagaactcaaacctctggaggaagtgctaaatttagctcaaagcaaaaactttcacttaagacccagggacttaatcagcaatatcaacgtaatagttctggaactaaagggatctgaaacaacattcatgtgtgaatatgctgatgagacagcaaccattgtagaatttctgaacagatggattacctttagtcaaagcatcatctcaacactgacttga

SEQ ID NO: 114 - DNA, 399 bp, Artificial Sequence
  IL-2 analog 8
cctacttcaagttctacaaagaaaacacagctacaactggagcatttactgctggatttacagatgattttgaatggaattaataattacaagaatcccaaactcaccaggatgctcacatttaagttttacatgcccaagaaggccacagaactgaaacatcttcagtgtctagaagaagaactcaaacctctggaggaagtgctaaatttagctcaaagctgtaactttcacttaagacccagggacttaatcagcaatatcaacgtaatagttctggaactaaagggatctgaaacaacattcatgtgtgaatatgctgatgagacagcaaccattgtagaatttctgaacagatggattacctttagtcaaagcatcatctcaacactgacttga

SEQ ID NO: 115 - DNA, 399 bp, Artificial Sequence
  IL-2 analog 9
cctacttcaagttctacaaagaaaacacagctacaactggagcatttactgctggatttacagatgattttgaatggaattaataattacaagaatcccaaactcaccgcgatgctcacatttaagttttacatgcccaagaaggccacagaactgaaacatcttcagtgtctagaagaagaactcaaacctctggaggaagtgctaaatttagctcaaagcaaaaactttcacttaagacccagggacttaatcagcaatatcaacgtaatagttctggaactaaagggatctgaaacaacattcatgtgtgaatatgctgatgagacagcaaccattgtagaatttctgaacagatggattacctttagtcaaagcatcatctcaacactgacttga

SEQ ID NO: 116 - DNA, 399 bp, Artificial Sequence
  IL-2 analog 10
cctacttcaagttctacaaagaaaacacagctacaactggagcatttactgctggatttacagatgattttgaatggaattaataattacaagaatcccaaactcaccaggatgctcacaaagaagttttacatgcccaagaaggccacagaactgaaacatcttcagtgtctagaagaagaactcaaacctctggaggaagtgctaaatttagctcaaagcaaaaactttcacttaagacccagggacttaatcagcaatatcaacgtaatagttctggaactaaagggatctgaaacaacattcatgtgtgaatatgctgatgagacagcaaccattgtagaatttctgaacagatggattacctttagtcaaagcatcatctcaacactgacttga

SEQ ID NO: 117 - DNA, 399 bp, Artificial Sequence
  IL-2 analog 11
cctacttcaagttctacaaagaaaacacagctacaactggagcatttactgctggatttacagatgattttgaatggaattaataattacaagaatcccaaactcaccaggatgctcacagctaagttttacatgcccaagaaggccacagaactgaaacatcttcagtgtctagaagaagaactcaaacctctggaggaagtgctaaatttagctcaaagcaaaaactttcacttaagacccagggacttaatcagcaatatcaacgtaatagttctggaactaaagggatctgaaacaacattcatgtgtgaatatgctgatgagacagcaaccattgtagaatttctgaacagatggattacctttagtcaaagcatcatctcaacactgacttga

SEQ ID NO: 118 - DNA, 399 bp, Artificial Sequence
  IL-2 analog 12
cctacttcaagttctacaaagaaaacacagctacaactggagcatttactgctggatttacagatgattttgaatggaattaataattacaagaatcccaaactcaccgcgatgctcacaaagaagttttacatgcccaagaaggccacagaactgaaacatcttcagtgtctagaagaagaactcaaacctctggaggaagtgctaaatttagctcaaagcaaaaactttcacttaagacccagggacttaatcagcaatatcaacgtaatagttctggaactaaagggatctgaaacaacattcatgtgtgaatatgctgatgagacagcaaccattgtagaatttctgaacagatggattacctttagtcaaagcatcatctcaacactgacttga

SEQ ID NO: 119 - DNA, 399 bp, Artificial Sequence
  IL-2 analog 13
cctacttcaagttctacaaagaaaacacagctacaactggagcatttactgctggatttacagatgattttgaatggaattaataattacaagaatcccaaactcaccgcgatgctcacagctaagttttacatgcccaagaaggccacagaactgaaacatcttcagtgtctagaagaagaactcaaacctctggaggaagtgctaaatttagctcaaagcaaaaactttcacttaagacccagggacttaatcagcaatatcaacgtaatagttctggaactaaagggatctgaaacaacattcatgtgtgaatatgctgatgagacagcaaccattgtagaatttctgaacagatggattacctttagtcaaagcatcatctcaacactgacttga

SEQ ID NO: 120 - DNA, 399 bp, Artificial Sequence
  IL-2 analog 14
cctacttcaagttctacaaagaaaacacagctacaactggagcatttactgtacgatttacagatgattttgaatggaattaataattacaagaatcccaaactcaccgcgatgctcacaaagaagttttacatgcccaagaaggccacagaactgaaacatcttcagtgtctagaagaagaactcaaacctctggaggaagtgctaaatttagctcaaagcaaaaactttcacttaagacccagggacttaatcagcaatatcaacgtaatagttctggaactaaagggatctgaaacaacattcatgtgtgaatatgctgatgagacagcaaccattgtagaatttctgaacagatggattacctttagtcaaagcatcatctcaacactgacttga

SEQ ID NO: 121 - DNA, 399 bp, Artificial Sequence
  IL-2 analog 15
cctacttcaagttctacaaagaaaacacagctacaactggagcatttactgctggatttacagatgattttgaatggaattaataattacaagaatcccaaactcaccgcgatgctcacaaagaagttttacatgcccaagaaggccacagaactgaaacatcttcagtgtctagaagaagaactcaaacctctggaggaagtgctaaatttagctcaaagcaaaaactttcacttaagacccagggagttaatcagcaatatcaacgtaatagttctggaactaaagggatctgaaacaacattcatgtgtgaatatgctgatgagacagcaaccattgtagaatttctgaacagatggattacctttagtcaaagcatcatctcaacactgacttga

SEQ ID NO: 122 - DNA, 399 bp, Artificial Sequence
  IL-2 analog 16
cctacttcaagttctacaaagaaaacacagctacaactggagcatttactgctggatttacagatgattttgaatggaattaataattacaagaatcccaaactcaccgcgatgctcacaaagaagttttacatgcccaagaaggccacagaactgaaacatcttcagtgtctagaagaagaactcaaacctctggaggaagtgctaaatttagctcaaagcaaaaactttcacttaagacccagggacttaatcagccaaatcaacgtaatagttctggaactaaagggatctgaaacaacattcatgtgtgaatatgctgatgagacagcaaccattgtagaatttctgaacagatggattacctttagtcaaagcatcatctcaacactgacttga

SEQ ID NO: 123 - DNA, 399 bp, Artificial Sequence
  IL-2 analog 17
cctacttcaagttctacaaagaaaacacagctacaactggagcatttactgctggatttacagatgattttgaatggaattaataattacaagaatcccaaactcaccgcgatgctcacaaagaagttttacatgcccaagaaggccacagaactgaaacatcttcagtgtctagaagaagaactcaaacctctggaggaagtgctaaatttagctcaaagcaaaaactttcacttaagacccagggacttaatcagcaatatcaacacaatagttctggaactaaagggatctgaaacaacattcatgtgtgaatatgctgatgagacagcaaccattgtagaatttctgaacagatggattacctttagtcaaagcatcatctcaacactgacttga

SEQ ID NO: 124 - DNA, 399 bp, Artificial Sequence
  IL-2 analog 18
cctacttcaagttctacaaagaaaacacagctacaactggagcatttactgctggatttacagatgattttgaatggaattaataattacaagaatcccaaactcaccgcgatgctcacaaagaagttttacatgcccaagaaggccacagaactgaaacatcttcagtgtctagaacaggaactcaaacctctggaggaagtgctaaatttagctcaaagcaaaaactttcacttaagacccagggacttaatcagcaatatcaacgtaatagttctggaactaaagggatctgaaacaacattcatgtgtgaatatgctgatgagacagcaaccattgtagaatttctgaacagatggattacctttagtcaaagcatcatctcaacactgacttga

SEQ ID NO: 125 - DNA, 399 bp, Artificial Sequence
  IL-2 analog 19
cctacttcaagttctacaaagaaaacacagctacaactggagcatttactgctggatttacagatgattttgaatggaattaataattacaagaatcccaaactcaccgcgatgctcacaaagaagttttacatgcccaagaaggccacagaactgaaacatcttcagtgtctagaagaagaactcaaacctctggaggaagtgctaaatttagctcaaagcaaaaactttcacttagaccccagggacttaatcagcaatatcaacgtatttgttctggaactaaagggatctgaaacaacattcatgtgtgaatatgctgatgagacagcaaccattgtagaatttctgaacagatggattacctttagtcaaagcatcatctcaacactgacttga

SEQ ID NO: 126 - DNA, 399 bp, Artificial Sequence
  IL-2 analog 20
cctacttcaagttctacaaagaaaacacagctacaactggagcatttactgctggatttacagatgattttgaatggaattaataattacaagaatcccaaactcaccgcgatgctcacaaagaagttttacatgcccaagaaggccacagaactgaaacatcttcagtgtctagaagaagaactcaaacctctggaggaagtgctaaatttagctcaaagcaaaaactttcacttaagacccagggacgtagtcagcaatatcaacgtatttgttctggaactaaagggatctgaaacaacattcatgtgtgaatatgctgatgagacagcaaccattgtagaatttctgaacagatggattacctttagtcaaagcatcatctcaacactgacttga

SEQ ID NO: 127 - DNA, 399 bp, Artificial Sequence
  IL-2 analog 21
cctacttcaagttctacaaagaaaacacagctacaactggagcatttactgctggatttacagatgattttgaatggaattaataattacaagaatcccaaactcaccgcgatgctcacaaagaagttttacatgcccaagaaggccacagaactgaaacatcttcagtgtctagaagaagaactcaaacctctggaggaagtgctaaatttagctcaaagcaaaaactttcactttgaccccagggacgtagtcagcaatatcaacgtatttgttctggaactaaagggatctgaaacaacattcatgtgtgaatatgctgatgagacagcaaccattgtagaatttctgaacagatggattacctttagtcaaagcatcatctcaacactgacttga

SEQ ID NO: 128 - DNA, 399 bp, Artificial Sequence
  IL-2 analog 22
cctacttcaagttctacaaagaaaacacaggtacaactggagcatttactgctggatttacagatgattttgaatggaattaataattacaagaatcccaaactcaccgcgatgctcacaaagaagttttacatgcccaagaaggccacagaactgaaacatcttcagtgtctagaagaagaactcaaacctctggaggaagtgctaaatttagctcaaagcaaaaactttcacttaagacccagggacttaatcagcaatatcaacgtaatagttctggaactaaagggatctgaaacaacattcatgtgtgaatatgctgatgagacagcaaccattgtagaatttctgaacagatggattacctttagtcaaagcatcatctcaacactgacttga

SEQ ID NO: 129 - DNA, 399 bp, Artificial Sequence
  IL-2 analog 23
cctacttcaagttctacaaagaaaacacagtttcaactggagcatttactgctggatttacagatgattttgaatggaattaataattacaagaatcccaaactcaccgcgatgctcacaaagaagttttacatgcccaagaaggccacagaactgaaacatcttcagtgtctagaagaagaactcaaacctctggaggaagtgctaaatttagctcaaagcaaaaactttcacttaagacccagggacttaatcagcaatatcaacgtaatagttctggaactaaagggatctgaaacaacattcatgtgtgaatatgctgatgagacagcaaccattgtagaatttctgaacagatggattacctttagtcaaagcatcatctcaacactgacttga

SEQ ID NO: 130 - DNA, 399 bp, Artificial Sequence
  IL-2 analog 24
cctacttcaagttctacaaagaaaacacagctacaactggagcatttactggtggatttacagatgattttgaatggaattaataattacaagaatcccaaactcaccgcgatgctcacaaagaagttttacatgcccaagaaggccacagaactgaaacatcttcagtgtctagaagaagaactcaaacctctggaggaagtgctaaatttagctcaaagcaaaaactttcacttaagacccagggacttaatcagcaatatcaacgtaatagttctggaactaaagggatctgaaacaacattcatgtgtgaatatgctgatgagacagcaaccattgtagaatttctgaacagatggattacctttagtcaaagcatcatctcaacactgacttga

SEQ ID NO: 131 - DNA, 399 bp, Artificial Sequence
  IL-2 analog 25
cctacttcaagttctacaaagaaaacacagctacaactggagcatttactgttcgatttacagatgattttgaatggaattaataattacaagaatcccaaactcaccgcgatgctcacaaagaagttttacatgcccaagaaggccacagaactgaaacatcttcagtgtctagaagaagaactcaaacctctggaggaagtgctaaatttagctcaaagcaaaaactttcacttaagacccagggacttaatcagcaatatcaacgtaatagttctggaactaaagggatctgaaacaacattcatgtgtgaatatgctgatgagacagcaaccattgtagaatttctgaacagatggattacctttagtcaaagcatcatctcaacactgacttga

SEQ ID NO: 132 - DNA, 399 bp, Artificial Sequence
  IL-2 analog 26
cctacttcaagttctacaaagaaaacacagctacaactggagcatttactgctggatttacagatgattttgaatggaattaataattacaagaatcccaaactcaccgcgatgctcacaaagaagttttacatgcccaagaaggccacagaactgaaacatcttcagtgtctagaagaagaactcaaacctctggaggaagtgctaaatttagctcaaagcaaaaactttcacttaagacccagggacttaatcagcaatttcaacgtaatagttctggaactaaagggatctgaaacaacattcatgtgtgaatatgctgatgagacagcaaccattgtagaatttctgaacagatggattacctttagtcaaagcatcatctcaacactgacttga

SEQ ID NO: 133 - DNA, 399 bp, Artificial Sequence
  IL-2 analog 27
cctacttcaagttctacaaagaaaacacagctacaactggagcatttactgctggatttacagatgattttgaatggaattaataattacaagaatcccaaactcaccgcgatgctcacaaagaagttttacatgcccaagaaggccacagaactgaaacatcttcagtgtctagaagaagaactcaaacctctggaggaagtgctaaatttagctcaaagcaaaaactttcacttaagacccagggacttaatcagcaatatcaactttatagttctggaactaaagggatctgaaacaacattcatgtgtgaatatgctgatgagacagcaaccattgtagaatttctgaacagatggattacctttagtcaaagcatcatctcaacactgacttga

SEQ ID NO: 134 - DNA, 399 bp, Artificial Sequence
  IL-2 analog 28
cctacttcaagttctacaaagaaaacacagctacaactggagcatttactgctggatttacagatgattttgaatggaattaataattacaagaatcccaaactcaccgcgatgctcacaaagaagttttacatgcccaagaaggccacagaactgaaacatcttcagtgtctagaagaagaactcaaacctctggaggaagtgctaaatttagctcaaagcaaaaactttcacttaagacccagggacttaatcagcaatatcaacgtaatagttgtggaactaaagggatctgaaacaacattcatgtgtgaatatgctgatgagacagcaaccattgtagaatttctgaacagatggattacctttagtcaaagcatcatctcaacactgacttga

SEQ ID NO: 135 - DNA, 399 bp, Artificial Sequence
  IL-2 analog 29
cctacttcaagttctacaaagaaaacacagctacaactggagcatttactgctggatttacagatgattttgaatggaattaataattacaagaatcccaaactcaccgcgatgctcacaaagaagttttacatgcccaagaaggccacagaactgaaacatcttcagtgtctagaagaagaactcaaacctctggaggaagtgctaaatttagctcaaagcaaaaactttcacttaagacccagggacttaatcagcaatatcaacgtaatagttctggaactaaagggatctgaaacaacattcatgtgtgaatatgctgatgagacagcaaccattgtagaatttctgaacagatggattacctttagtacaagcatcatctcaacactgacttga

SEQ ID NO: 136 - DNA, 399 bp, Artificial Sequence
  IL-2 analog 30
cctacttcaagttctacaaagaaaacacagctacaactggagcatttactgctggatttacagatgattttgaatggaattaataattacaagaatcccaaactcaccgcgatgctcacatttaagttttacatgcccaagaaggccacagaactgaaacatcttcagtgtctagaagaagaactcaaacctctggaggaagtgctaaatttagctcaaagcaaaaactttcacttagaccccagggacttaatcagcaatatcaacgtatttgttctggaactaaagggatctgaaacaacattcatgtgtgaatatgctgatgagacagcaaccattgtagaatttctgaacagatggattacctttagtcaaagcatcatctcaacactgacttga

SEQ ID NO: 137 - DNA, 399 bp, Artificial Sequence
  IL-2 analog 31
cctacttcaagttctacaaagaaaacacagctacaactggagcatttactgctggatttacagatgattttgaatggaattaataattacaagaatcccaaactcaccgcgatgctcacatttaagttttacatgcccaagaaggccacagaactgaaacatcttcagtgtctagaagaagaactcaaacctctggaggaagtgctaaatttagctcaaagcaaaaactttcacttaagacccagggagttaatcagcaatatcaacgtaatagttctggaactaaagggatctgaaacaacattcatgtgtgaatatgctgatgagacagcaaccattgtagaatttctgaacagatggattacctttagtcaaagcatcatctcaacactgacttga

SEQ ID NO: 138 - DNA, 399 bp, Artificial Sequence
  IL-2 analog 32
cctacttcaagttctacaaagaaaacacagctacaactggagcatttactgctggatttacagatgattttgaatggaattaataattacaagaatcccaaactcaccgcgatgctcacatttaagttttacatgcccaagaaggccacagaactgaaacatcttcagtgtctagaagaagaactcaaacctctggaggaagtgctaaatttagctcaaagcaaaaactttcacttagaccccagggagttaatcagcaatatcaacgtatttgttctggaactaaagggatctgaaacaacattcatgtgtgaatatgctgatgagacagcaaccattgtagaatttctgaacagatggattacctttagtcaaagcatcatctcaacactgacttga

SEQ ID NO: 139 - DNA, 399 bp, Artificial Sequence
  IL-2 analog 33
cctacttcaagttctacaaagaaaacacagctacaactggagcatttactgctggatttacagatgattttgaatggaattaataattacaagaatcccaaactcaccgcgatgctcacatttaagttttacatgcccaagaaggccacagaactgaaacatcttcagtgtctagaagaagaactcaaacctctggaggaagtgctaaatttagctcaaagcaaaaactttcactttagacccagggacttaatcagcaatatcaacgtaatagttctggaactaaagggatctgaaacaacattcatgtgtgaatatgctgatgagacagcaaccattgtagaatttctgaacagatggattacctttagtcaaagcatcatctcaacactgacttga

SEQ ID NO: 140 - DNA, 399 bp, Artificial Sequence
  IL-2 analog 34
cctacttcaagttctacaaagaaaacacagctacaactggagcatttactgctggatttacagatgattttgaatggaattaataattacaagaatcccaaactcaccgcgatgctcacatttaagttttacatgcccaagaaggccacagaactgaaacatcttcagtgtctagaagaagaactcaaacctctggaggaagtgctaaatttagctcaaagcaaaaactttcactttagacccagggagttaatcagcaatatcaacgtaatagttctggaactaaagggatctgaaacaacattcatgtgtgaatatgctgatgagacagcaaccattgtagaatttctgaacagatggattacctttagtcaaagcatcatctcaacactgacttga

SEQ ID NO: 141 - DNA, 399 bp, Artificial Sequence
  IL-2 analog 35
cctacttcaagttctacaaagaaaacacagctacaactggagcatttactgctggatttacagatgattttgaatggaattaataattacaagaatcccaaactcaccgcgatgctcacatttaagttttacatgcccaagaaggccacagaactgaaacatcttcagtgtctagaagaagaactcaaacctctggaggaagtgctaaatttagctcaaagcaaaaactttcacttaagacccagggacttaatcagcaatatcaacgtaatagttttcgaatttaagggatctgaaacaacattcatgtgtgaatatgctgatgagacagcaaccattgtagaatttctgaacagatggattacctttagtcaaagcatcatctcaacactgacttga

SEQ ID NO: 142 - DNA, 399 bp, Artificial Sequence
  IL-2 analog 36
cctacttcaagttctacaaagaaaacacagctacaactggagcatttactgctggatttacagatgattttgaatggaattaataattacaagaatcccaaactcaccgcgatgctcacatttaagttttacatgcccaagaaggccacagaactgaaacatcttcagtgtctagaagaagaactcaaacctctggaggaagtgctaaatttagctcaaagcaaaaactttcacttaagacccagggacttaatcagcaatatcaacgtaatagttttcgaagtaaagggatctgaaacaacattcatgtgtgaatatgctgatgagacagcaaccattgtagaatttctgaacagatggattacctttagtcaaagcatcatctcaacactgacttga

SEQ ID NO: 143 - DNA, 399 bp, Artificial Sequence
  IL-2 analog 37
cctacttcaagttctacaaagaaaacacagctacaactggagcatttactgctggatttacagatgattttgaatggaattaataattacaagaatcccaaactcaccgcgatgctcacaaagaagttttacatgcccaagaaggccacagaactgaaacatcttcagtgtctagaagaagaactcaaacctctggaggaagtgctaaatttagctcaaagcaaaaactttcacttagaccccagggacttaatcagcaatatcaacgtattagttctggaactaaagggatctgaaacaacattcatgtgtgaatatgctgatgagacagcaaccattgtagaatttctgaacagatggattacctttagtcaaagcatcatctcaacactgacttga

SEQ ID NO: 144 - DNA, 399 bp, Artificial Sequence
  IL-2 analog 38
cctacttcaagttctacaaagaaaacacagctacaactggagcatttactgctggatttacagatgattttgaatggaattaataattacaagaatcccaaactcaccgcgatgctcacaaagaagttttacatgcccaagaaggccacagaactgaaacatcttcagtgtctagaagaagaactcaaacctctggaggaagtgctaaatttagctcaaagcaaaaactttcacttagaccccagggacttaatcagcaatatcaacgtatttgttttcgaatttaagggatctgaaacaacattcatgtgtgaatatgctgatgagacagcaaccattgtagaatttctgaacagatggattacctttagtcaaagcatcatctcaacactgacttga

SEQ ID NO: 145 - DNA, 399 bp, Artificial Sequence
  IL-2 analog 39
cctacttcaagttctacaaagaaaacacagctacaactggagcatttactgctggatttacagatgattttgaatggaattaataattacaagaatcccaaactcaccgcgatgctcacaaagaagttttacatgcccaagaaggccacagaactgaaacatcttcagtgtctagaagaagaactcaaacctctggaggaagtgctaaatttagctcaaagcaaaaactttcacttagaccccagggacttaatcagcaatatcaacgtatttgttttcgaagtaaagggatctgaaacaacattcatgtgtgaatatgctgatgagacagcaaccattgtagaatttctgaacagatggattacctttagtcaaagcatcatctcaacactgacttga

SEQ ID NO: 146 - DNA, 399 bp, Artificial Sequence
  IL-2 analog 40
cctacttcaagttctacaaagaaaacacagctacaactggagcatttactgctggatttacagatgattttgaatggaattaataattacaagaatcccaaactcaccgcgatgctcacaaagaagttttacatgcccaagaaggccacagaactgaaacatcttcagtgtctagaagaagaactcaaacctctggaggaagtgctaaatttagctcaaagcaaaaactttcacttagaccccagggacttaatcagcaatatcaacgtatttgttttcgaaattaagggatctgaaacaacattcatgtgtgaatatgctgatgagacagcaaccattgtagaatttctgaacagatggattacctttagtcaaagcatcatctcaacactgacttga

SEQ ID NO: 147 - DNA, 399 bp, Artificial Sequence
  IL-2 analog 41
cctacttcaagttctacaaagaaaacacagctacaactggagcatttactgctggatttacagatgattttgaatggaattaataattacaagaatcccaaactcaccaggatgctcacatttaagttttacatgcccaagaaggccacagaactgaaacatcttcagtgtctagaagaagaactcaaacctctggaggaagtgctaaatttagctcaaagcaaaaactttcactttgaccccagggacgtagtcagcaatatcaacgtatttgttctggaactaaagggatctgaaacaacattcatgtgtgaatatgctgatgagacagcaaccattgtagaatttctgaacagatggattacctttagtcaaagcatcatctcaacactgacttga

SEQ ID NO: 148 - DNA, 399 bp, Artificial Sequence
  IL-2 analog 42
cctacttcaagttctacaaagaaaacacagctacaactggagcatttactgctggatttacagatgattttgaatggaattaataattacaagaatcccaaactcaccgcgatgctcacaaagaagttttacatgcccaagaaggccacagaactgaaacatcttcagtgtctagaagaagaactcaaacctctggaggaagtgctaaatttagctcaaagcaaaaactttcacttagaacccagggacttaatcagcaatatcaacgtatttgttctggaactaaagggatctgaaacaacattcatgtgtgaatatgctgatgagacagcaaccattgtagaatttctgaacagatggattacctttagtcaaagcatcatctcaacactgacttga

SEQ ID NO: 149 - DNA, 399 bp, Artificial Sequence; identical to SEQ ID NO: 143
  IL-2 analog 43

SEQ ID NO: 150 - DNA, 399 bp, Artificial Sequence
  IL-2 analog 44
cctacttcaagttctacaaagaaaacacagctacaactggagcatttactgctggatttacagatgattttgaatggaattaataattacaagaatcccaaactcaccgcgatgctcacaaagaagttttacatgcccaagaaggccacagaactgaaacatcttcagtgtctagaagaagaactcaaacctctggaggaagtgctaaatttagctcaaagcaaaaactttcacttagaccccagggtcttaatcagcaatatcaacgtatttgttctggaactaaagggatctgaaacaacattcatgtgtgaatatgctgatgagacagcaaccattgtagaatttctgaacagatggattacctttagtcaaagcatcatctcaacactgacttga

SEQ ID NO: 151 - DNA, 399 bp, Artificial Sequence
  IL-2 analog 45
cctacttcaagttctacaaagaaaacacagctacaactggagcatttactgctggatttacagatgattttgaatggaattaataattacaagaatcccaaactcaccgcgatgctcacaaagaagttttacatgcccaagaaggccacagaactgaaacatcttcagtgtctagaagaagaactcaaacctctggaggaagtgctaaatttagctcaaagcaaaaactttcacttagaccccaggttcttaatcagcaatatcaacgtatttgttctggaactaaagggatctgaaacaacattcatgtgtgaatatgctgatgagacagcaaccattgtagaatttctgaacagatggattacctttagtcaaagcatcatctcaacactgacttga

SEQ ID NO: 152 - DNA, 399 bp, Artificial Sequence
  IL-2 analog 46
cctacttcaagttctacaaagaaaacacagctacaactggagcatttactgctggttttacagatgattttgaatggaattaataattacaagaatcccaaactcaccgcgatgctcacaaagaagttttacatgcccaagaaggccacagaactgaaacatcttcagtgtctagaagaagaactcaaacctctggaggaagtgctaaatttagctcaaagcaaaaactttcacttagaccccagggacttaatcagcaatatcaacgtatttgttctggaactaaagggatctgaaacaacattcatgtgtgaatatgctgatgagacagcaaccattgtagaatttctgaacagatggattacctttagtcaaagcatcatctcaacactgacttga

SEQ ID NO: 153 - DNA, 399 bp, Artificial Sequence
  IL-2 analog 47
cctacttcaagttctacaaagaaaacacagctacaactggagcatttactgctgtttttacagatgattttgaatggaattaataattacaagaatcccaaactcaccgcgatgctcacaaagaagttttacatgcccaagaaggccacagaactgaaacatcttcagtgtctagaagaagaactcaaacctctggaggaagtgctaaatttagctcaaagcaaaaactttcacttagaccccagggacttaatcagcaatatcaacgtatttgttctggaactaaagggatctgaaacaacattcatgtgtgaatatgctgatgagacagcaaccattgtagaatttctgaacagatggattacctttagtcaaagcatcatctcaacactgacttga

SEQ ID NO: 154 - DNA, 399 bp, Artificial Sequence
  IL-2 analog 48
cctacttcaagttctacaaagaaaacacagctacaactggagcatttactgctggatttacagatgattttgaatggaattaataattacaagaatcccaaactcaccgcgatgctcacaaagaagttttacatgcccaagaaggccacagaactgaaacatcttcagtgtctagaagaagaactcaaacctctggaggaagtgctaaatttagctcaaagcaaaaactttcacttagaccccagggacttaatcagcgttatcaacgtatttgttctggaactaaagggatctgaaacaacattcatgtgtgaatatgctgatgagacagcaaccattgtagaatttctgaacagatggattacctttagtcaaagcatcatctcaacactgacttga

SEQ ID NO: 155 - DNA, 399 bp, Artificial Sequence
  IL-2 analog 49
cctacttcaagttctacaaagaaaacacagctacaactggagcatttactgctggatttacagatgattttgaatggaattaataattacaagaatcccaaactcaccgcgatgctcacaaagaagttttacatgcccaagaaggccacagaactgaaacatcttcagtgtctagaagaagaactcaaacctctggaggaagtgctaaatttagctcaaagcaaaaactttcacttagaccccagggacttaatcagctttatcaacgtatttgttctggaactaaagggatctgaaacaacattcatgtgtgaatatgctgatgagacagcaaccattgtagaatttctgaacagatggattacctttagtcaaagcatcatctcaacactgacttga

SEQ ID NO: 156 - DNA, 399 bp, Artificial Sequence
  IL-2 analog 50
cctacttcaagttctacaaagaaaacacagctacaactggagcatttactgctggatttacagatgattttgaatggaattaataattacaagaatcccaaactcaccaggatgctcacaaagaagttttacatgcccaagaaggccacagaactgaaacatcttcagtgtctagaagaagaactcaaacctctggaggaagtgctaaatttagctcaaagcaaaaactttcactttgaccccagggacgtagtcagcaatatcaacgtatttgttctggaactaaagggatctgaaacaacattcatgtgtgaatatgctgatgagacagcaaccattgtagaatttctgaacagatggattacctttagtcaaagcatcatctcaacactgacttga

SEQ ID NO: 157 - DNA, 399 bp, Artificial Sequence
  IL-2 analog 51
cctacttcaagttctacaaagaaaacacagctacaactggagcatttactgctggatttacagatgattttgaatggaattaataattacaagaatcccaaactcaccaggatgctcacatttaagttttacatgcccaagaaggccacagaactgaaacatcttcagtgtctagaacaggaactcaaacctctggaggaagtgctaaatttagctcaaagcaaaaactttcacttagaccccagggacttaatcagcaatatcaacgtatttgttctggaactaaagggatctgaaacaacattcatgtgtgaatatgctgatgagacagcaaccattgtagaatttctgaacagatggattacctttagtcaaagcatcatctcaacactgacttga

SEQ ID NO: 158 - DNA, 399 bp, Artificial Sequence
  IL-2 analog 52
cctacttcaagttctacaaagaaaacacagctacaactggagcatttactgctggatttacagatgattttgaatggaattaataattacaagaatcccaaactcaccgcgatgctcacaaagaagttttacatgcccaagaaggccacagaactgaaacatcttcagtgtctagaagaagaactcaaacctctggaggaagtgctaaatttagctcaaagcaaaaactttcactttgaccccagggacttaatcagcaatatcaacgtatttgttctggaactaaagggatctgaaacaacattcatgtgtgaatatgctgatgagacagcaaccattgtagaatttctgaacagatggattacctttagtcaaagcatcatctcaacactgacttga

SEQ ID NO: 159 - DNA, 399 bp, Artificial Sequence
  IL-2 analog 53
cctacttcaagttctacaaagaaaacacagctacaactggagcatttactgctggatttacagatgattttgaatggaattaataattacaagaatcccaaactcaccgcgatgctcacaaagaagttttacatgcccaagaaggccacagaactgaaacatcttcagtgtctagaagaagaactcaaacctctggaggaagtgctaaatttagctcaaagcaaaaactttcactttgaccccagggagttaatcagcaatatcaacgtatttgttctggaactaaagggatctgaaacaacattcatgtgtgaatatgctgatgagacagcaaccattgtagaatttctgaacagatggattacctttagtcaaagcatcatctcaacactgacttga

SEQ ID NO: 160 - DNA, 399 bp, Artificial Sequence
  IL-2 analog 54
cctacttcaagttctacaaagaaaacacagctacaactggagcatttactgctggatttacagatgattttgaatggaattaataattacaagaatcccaaactcaccgcgatgctcacaaagaagttttacatgcccaagaaggccacagaactgaaacatcttcagtgtctagaagaagaactcaaacctctggaggaagtgctaaatttagctcacagcaaaaactttcacttagaccccagggacttaatcagcaatatcaacgtatttgttctggaactaaagggatctgaaacaacattcatgtgtgaatatgctgatgagacagcaaccattgtagaatttctgaacagatggattacctttagtcaaagcatcatctcaacactgacttga

SEQ ID NO: 161 - DNA, 399 bp, Artificial Sequence
  IL-2 analog 55
cctacttcaagttctacaaagaaaacacagctacaactggagcatttactgctggatttacagatgattttgaatggaattaataattacaagaatcccaaactcaccgcgatgctcacaaagaagttttacatgcccaagaaggccacagaactgaaacatcttcagtgtctagaagaagaactcaaacctctggaggaagtgctaaatttagctcacagcaaaaactttcactttgaccccagggacttaatcagcaatatcaacgtatttgttctggaactaaagggatctgaaacaacattcatgtgtgaatatgctgatgagacagcaaccattgtagaatttctgaacagatggattacctttagtcaaagcatcatctcaacactgacttga

SEQ ID NO: 162 - DNA, 399 bp, Artificial Sequence
  IL-2 analog 56
cctacttcaagttctacaaagaaaacacagctacaactggagcatttactgctggatttacagatgattttgaatggaattaataattacaagaatcccaaactcaccgcgatgctcacaaagaagtttgccatgcccaagaaggccacagaactgaaacatcttcagtgtctagaagaagaactcaaacctctggaggaagtgctaaatttagctcacagcaaaaactttcacttagaccccagggacttaatcagcaatatcaacgtatttgttctggaactaaagggatctgaaacaacattcatgtgtgaatatgctgatgagacagcaaccattgtagaatttctgaacagatggattacctttagtcaaagcatcatctcaacactgacttga

SEQ ID NO: 163 - DNA, 399 bp, Artificial Sequence
  IL-2 analog 57
cctacttcaagttctacaaagaaaacacagctacaactggagcatttactgctggatttacagatgattttgaatggaattaataattacaagaatcccaaactcaccgcgatgctcacaaagaagtttgccatgcccaagaaggccacagaactgaaacatcttcagtgtctagaagaagaactcaaacctctggaggaagtgctaaatttagctcacagcaaaaactttcactttgaccccagggacttaatcagcaatatcaacgtatttgttctggaactaaagggatctgaaacaacattcatgtgtgaatatgctgatgagacagcaaccattgtagaatttctgaacagatggattacctttagtcaaagcatcatctcaacactgacttga

SEQ ID NO: 164 - DNA, 399 bp, Artificial Sequence
  IL-2 analog 58
cctacttcaagttctacaaagaaaacacagctacaactggagcatttactgctggatttacagatgattttgaatggaattaataattacaagaatcccaaactcaccgcgatgctcacaaagaagttttacatgcccaagaaggccacagaactgaaacatcttcagtgtctagaagaagaactcaaacctctggaggaagtgctaaatttagctcaaagcaaaaactttcactttgaccccagggacgctgccagcaatatcaacgtatttgttctggaactaaagggatctgaaacaacattcatgtgtgaatatgctgatgagacagcaaccattgtagaatttctgaacagatggattacctttagtcaaagcatcatctcaacactgacttga

SEQ ID NO: 165 - DNA, 399 bp, Artificial Sequence
  IL-2 analog 59
cctacttcaagttctacaaagaaaacacagctacaactggagcatttactgctggatttacagatgattttgaatggaattaataattacaagaatcccaaactcaccgcgatgctcacaaagaagttttacatgcccaagaaggccacagaactgaaacatcttcagtgtctagaagaagaactcaaacctctggaggaagtgctaaatttagctcaaagcaaaaactttcactttgaccccagggacgctgccagcaatatcaacgtatatgttctggaactaaagggatctgaaacaacattcatgtgtgaatatgctgatgagacagcaaccattgtagaatttctgaacagatggattacctttagtcaaagcatcatctcaacactgacttga

SEQ ID NO: 166 - DNA, 399 bp, Artificial Sequence
  IL-2 analog 60
cctacttcaagttctacaaagaaaacacagctacaactggagcatttactgctggatttacagatgattttgaatggaattaataattacaagaatcccaaactcaccgcgatgctcacaaagaagtttgccatgcccaagaaggccacagaactgaaacatcttcagtgtctagaagaagaactcaaacctctggaggaagtgctaaatttagctcaaagcaaaaactttcactatagacccagggacgctgccagcaatatcaacgtatatgttctggaactaaagggatctgaaacaacattcatgtgtgaatatgctgatgagacagcaaccattgtagaatttctgaacagatggattacctttagtcaaagcatcatctcaacactgacttga

SEQ ID NO: 167 - DNA, 399 bp, Artificial Sequence
  IL-2 analog 61
cctacttcaagttctacaaagaaaacacagctacaactggagcatttactgctggatttacagatgattttgaatggaattaataattacaagaatcccaaactcaccgcgatgctcacaaagaagttttacatgcccaagaaggccacagaactgaaacatcttcagtgtctagaagaagaactcaaacctctggaggaagtgctaaatttagctcaaagcaaaaactttcactatgaccccagggacggtgttagcaatatcaacgtatatgttctggaactaaagggatctgaaacaacattcatgtgtgaatatgctgatgagacagcaaccattgtagaatttctgaacagatggattacctttagtcaaagcatcatctcaacactgacttga

SEQ ID NO: 168 - DNA, 399 bp, Artificial Sequence
  IL-2 analog 62
cctacttcaagttctacaaagaaaacacagctacaactggagcatttactgctggatttacagatgattttgaatggaattaataattacaagaatcccaaactcaccgcgatgctcacaaagaagttttacatgcccaagaaggccacagaactgaaacatcttcagtgtctagaagaagaactcaaacctctggaggaagtgctaaatttagctcaaagcaaaaactttcactgggaacccagggacggagccagcaatatcaacgtatttgttctggaactaaagggatctgaaacaacattcatgtgtgaatatgctgatgagacagcaaccattgtagaatttctgaacagatggattacctttagtcaaagcatcatctcaacactgacttga

SEQ ID NO: 169 - DNA, 399 bp, Artificial Sequence
  IL-2 analog 63
cctacttcaagttctacaaagaaaacacagctacaactggagcatttactgctggatttacagatgattttgaatggaattaataattacaagaatcccaaactcaccgcgatgctcacaaagaagttttacatgcccaagaaggccacagaactgaaacatcttcagtgtctagaagaagaactcaaacctctggaggaagtgctaaatttagctcaaagcaaaaactttcacgacgaacccagggacacaggcagcaatatcaacgtatttgttctggaactaaagggatctgaaacaacattcatgtgtgaatatgctgatgagacagcaaccattgtagaatttctgaacagatggattacctttagtcaaagcatcatctcaacactgacttga

SEQ ID NO: 170 - DNA, 399 bp, Artificial Sequence
  IL-2 analog 64
cctacttcaagttctacaaagaaaacacagctacaactggagcatttactgctggatttacagatgattttgaatggaattaataattacaagaatcccaaactcaccgcgatgctcacaaagaagttttacatgcccaagaaggccacagaactgaaacatcttcagtgtctagaagaagaactcaaacctctggaggaagtgctaaatttagctcaaagcaaaaactttcactacaaccccagggacgtagtcagcaatatcaacgtatttgttctggaactaaagggatctgaaacaacattcatgtgtgaatatgctgatgagacagcaaccattgtagaatttctgaacagatggattacctttagtcaaagcatcatctcaacactgacttga

SEQ ID NO: 171 - DNA, 399 bp, Artificial Sequence
  IL-2 analog 65
cctacttcaagttctacaaagaaaacacagctacaactggagcatttactgctggatttacagatgattttgaatggaattaataattacaagaatcccaaactcaccgcgatgctcacaaagaagttttacatgcccaagaaggccacagaactgaaacatcttcagtgtctagaagaagaactcaaacctctggaggaagtgctaaatttagctcaaagcaaaaactttcactacgaacccagggacgtagtcagcaatatcaacgtatttgttctggaactaaagggatctgaaacaacattcatgtgtgaatatgctgatgagacagcaaccattgtagaatttctgaacagatggattacctttagtcaaagcatcatctcaacactgacttga

SEQ ID NO: 172 - DNA, 399 bp, Artificial Sequence
  IL-2 analog 66
cctacttcaagttctacaaagaaaacacagctacaactggagcatttactgctggatttacagatgattttgaatggaattaataattacaagaatcccaaactcaccgcgatgctcacaaagaagttttacatgcccaagaaggccacagaactgaaacatcttcagtgtctagaagaagaactcaaacctctggaggaagtgctaaatttagctcaaagcaaaaactttcacttcgaacccagggacttcgtcagcaatatcaacgtatttgttctggaactaaagggatctgaaacaacattcatgtgtgaatatgctgatgagacagcaaccattgtagaatttctgaacagatggattacctttagtcaaagcatcatctcaacactgacttga

SEQ ID NO: 173 - DNA, 399 bp, Artificial Sequence
  IL-2 analog 67
cctacttcaagttctacaaagaaaacacagctacaactggagcatttactgctggatttacagatgattttgaatggaattaataattacaagaatcccaaactcaccgcgatgctcacaaagaagttttacatgcccaagaaggccacagaactgaaacatcttcagtgtctagaagaagaactcaaacctctggaggaagtgctaaatttagctcaaagcaaaaactttcactatgaccccagggacttcgtcagcaatatcaacgtatgggttctggacctaaagggatctgaaacaacattcatgtgtgaatatgctgatgagacagcaaccattgtagaatttctgaacagatggattacctttagtcaaagcatcatctcaacactgacttga

SEQ ID NO: 174 - DNA, 399 bp, Artificial Sequence
  IL-2 analog 68
cctacttcaagttctacaaagaaaacacagctacaactggagcatttactgctggatttacagatgattttgaatggaattaataattacaagaatcccaaactcaccgcgatgctcacaaagaagttttacatgcccaagaaggccacagaactgaaacatcttcagtgtctagaagaagaactcaaacctctggaggaagtgctaaatttagctcaaagcaaaaactttcacttcgaacccagggacatagtcagcaatatcaacgaattcgttctggaactaaagggatctgaaacaacattcatgtgtgaatatgctgatgagacagcaaccattgtagaatttctgaacagatggattacctttagtcaaagcatcatctcaacactgacttga

SEQ ID NO: 175 - DNA, 399 bp, Artificial Sequence
  IL-2 analog 69
cctacttcaagttctacaaagaaaacacagctacaactggagcatttactgctggatttacagatgattttgaatggaattaataattacaagaatcccaaactcaccgcgatgctcacaaagaagttttacatgcccaagaaggccacagaactgaaacatcttcagtgtctagaagaagaactcaaacctctggaggaagtgctaaatttagctcaaagcaaaaactttcactacgaacccagggacttcctcagcaatatcaacgaatgggttctggacctaaagggatctgaaacaacattcatgtgtgaatatgctgatgagacagcaaccattgtagaatttctgaacagatggattacctttagtcaaagcatcatctcaacactgacttga

SEQ ID NO: 176 - DNA, 399 bp, Artificial Sequence
  IL-2 analog 70
cctacttcaagttctacaaagaaaacacagctacaactggagcatttactgctggatttacagatgattttgaatggaattaataattacaagaatcccaaactcaccgcgatgctcacaaagaagttttacatgcccaagaaggccacagaactgaaacatcttcagtgtctagaagaagaactcaaacctctggaggaagtgctaaatttagctcaaagcaaaaactttcactatgaccccagggacgtagtcagcaatatcaacgtatttgttctggaactaaagggatctgaaacaacattcatgtgtgaatatgctgatgagacagcaaccattgtagaatttctgaacagatggattacctttagtcaaagcatcatctcaacactgacttga

SEQ ID NO: 177 - DNA, 399 bp, Artificial Sequence
  IL-2 analog 71
cctacttcaagttctacaaagaaaacacagctacaactggagcatttactgctggatttacagatgattttgaatggaattaataattacaagaatcccaaactcaccgcgatgctcacaaagaagttttacatgcccaagaaggccacagaactgaaacatcttcagtgtctagaagaagaactcaaacctctggaggaagtgctaaatttagctcaaagcaaaaactttcacttcgaacccagggacgtagtcagcaatatcaacgtatttgttctggaactaaagggatctgaaacaacattcatgtgtgaatatgctgatgagacagcaaccattgtagaatttctgaacagatggattacctttagtcaaagcatcatctcaacactgacttga

SEQ ID NO: 178 - DNA, 399 bp, Artificial Sequence
  IL-2 analog 72
cctacttcaagttctacaaagaaaacacagctacaactggagcatttactgctggatttacagatgattttgaatggaattaataattacaagaatcccaaactcaccgcgatgctcacaaagaagttttacatgcccaagaaggccacagaactgaaacatcttcagtgtctagaagaagaactcaaacctctggaggaagtgctaaatttagctcaaagcaaaaactttcactttgaccccagggacgtaggcagcaatatcaacgtatttgttctggaactaaagggatctgaaacaacattcatgtgtgaatatgctgatgagacagcaaccattgtagaatttctgaacagatggattacctttagtcaaagcatcatctcaacactgacttga

SEQ ID NO: 179 - DNA, 399 bp, Artificial Sequence
  IL-2 analog 73
cctacttcaagttctacaaagaaaacacagctacaactggagcatttactgctggatttacagatgattttgaatggaattaataattacaagaatcccaaactcaccgcgatgctcacaaagaagttttacatgcccaagaaggccacagaactgaaacatcttcagtgtctagaagaagaactcaaacctctggaggaagtgctaaatttagctcaaagcaaaaactttcactttgaccccagggactgggtcagcaatatcaacgtatttgttctggaactaaagggatctgaaacaacattcatgtgtgaatatgctgatgagacagcaaccattgtagaatttctgaacagatggattacctttagtcaaagcatcatctcaacactgacttga

SEQ ID NO: 180 - DNA, 399 bp, Artificial Sequence
  IL-2 analog 74
cctacttcaagttctacaaagaaaacacagctacaactggagcatttactgctggatttacagatgattttgaatggaattaataattacaagaatcccaaactcaccgatatgctcacaaagaagttttacatgcccaagaaggccacagaactgaaacatcttcagtgtctagaagaagaactcaaacctctggaggaagtgctaaatttagctcaaagcaaaaactttcactatgaccccagggacgtagtcagcaatatcaacgtatttgttctggaactaaagggatctgaaacaacattcatgtgtgaatatgctgatgagacagcaaccattgtagaatttctgaacagatggattacctttagtcaaagcatcatctcaacactgacttga

SEQ ID NO: 181 - DNA, 399 bp, Artificial Sequence
  IL-2 analog 75
cctacttcaagttctacaaagaaaacacagctacaactggagcatttactgctggatttacagatgattttgaatggaattaataattacaagaatcccaaactcaccgcgatgctcacaaagaagtttgccatgcccaagaaggccacagaactgaaacatcttcagtgtctagaagaagaactcaaacctctggaggaagtgctaaatttagctcaaagcaaaaactttcacttcgaacccagggacgtagtcagcaatatcaacgtatttgttctggaactaaagggatctgaaacaacattcatgtgtgaatatgctgatgagacagcaaccattgtagaatttctgaacagatggattacctttagtcaaagcatcatctcaacactgacttga

SEQ ID NO: 182 - DNA, 399 bp, Artificial Sequence
  IL-2 analog 76
cctacttcaagttctacaaagaaaacacagctacaactggagcatttactgctggatttacagatgattttgaatggaattaataattacaagaatcccaaactcaccgcgatgctcacaaagcagttttacatgcccaagaaggccacagaactgaaacatcttcagtgtctagaacgggaactcaaacctctggaggaagtgctaaatttagctcaaagcaaaaactttcactttgaccccagggacgtaggcagcaatatcaacgtatttgttctggaactaaagggatctgaaacaacattcatgtgtgaatatgctgatgagacagcaaccattgtagaatttctgaacagatggattacctttagtcaaagcatcatctcaacactgacttga

SEQ ID NO: 183 - DNA, 399 bp, Artificial Sequence
  IL-2 analog 77
cctacttcaagttctacaaagaaaacacagctacaactggagcatttactgctggatttacagatgattttgaatggaattaataattacaagaatcccaaactcaccgcgatgctcacaaaggagttttacatgcccaagaaggccacagaactgaaacatcttcagtgtctagaacgggaactcaaacctctggaggaagtgctaaatttagctcaaagcaaaaactttcactttgaccccagggactgggtcagcaatatcaacgtatttgttctggaactaaagggatctgaaacaacattcatgtgtgaatatgctgatgagacagcaaccattgtagaatttctgaacagatggattacctttagtcaaagcatcatctcaacactgacttga

SEQ ID NO: 184 - DNA, 399 bp, Artificial Sequence
  IL-2 analog 78
cctacttcaagttctacaaagaaaacacagctacaactggagcatttactgctggatttacagatgattttgaatggaattaataattacaagaatcccgaactcaccgcgatgctcacaaagaagttttacatgcccaagaaggccacagaactgaaacatcttcagtgtctagaagaagaactcaaacctctggaggaagtgctaaatttagctcaaagcaaaaactttcacttcgaacccagggacgtagtcagcaatatcaacgtatttgttctggaactaaagggatctgaaacaacattcatgtgtgaatatgctgatgagacagcaaccattgtagaatttctgaacagatggattacctttagtcaaagcatcatctcaacactgacttga

SEQ ID NO: 185 - DNA, 399 bp, Artificial Sequence
  IL-2 analog 79
cctacttcaagttctacaaagaaaacacagctacaactggagcatttactgctggatttacagatgattttgaatggaattaataattacaagaatcccgaactcaccgcgatgctcacaaagaagttttacatgcccaagaaggccacagaactgaaacatcttcagtgtctagaagaagaactcaaacctctggaggaagtgctaaatttagctcacagcaaaaactttcacttcgaacccagggacgtagtcagcaatatcaacgtatttgttctggaactaaagggatctgaaacaacattcatgtgtgaatatgctgatgagacagcaaccattgtagaatttctgaacagatggattacctttagtcaaagcatcatctcaacactgacttga

SEQ ID NO: 186 - DNA, 399 bp, Artificial Sequence
  IL-2 analog 80
cctacttcaagttctacaaagaaaacacagctacaactggagcatttactgctggatttacagatgattttgaatggaattaataattacaagaatcccgaactcaccgcgatgctcacaaagaagttttacatgcccaagaaggccacagaactgaaacatcttcagtgtctagaagaagaactcaaacctctggaggaagtgctaaatttagctcacagcaaaaactttcacttcgaaggcagggacgtagtcagcaatatcaacgtatttgttctggaactaaagggatctgaaacaacattcatgtgtgaatatgctgatgagacagcaaccattgtagaatttctgaacagatggattacctttagtcaaagcatcatctcaacactgacttga

SEQ ID NO: 187 - DNA, 399 bp, Artificial Sequence
  IL-2 analog 81
cctacttcaagttctacaaagaaaacacagctacaactggagcatttactgctggatttacagatgattttgaatggaattaataattacaagaatcccgaactcaccgcgatgctcacaaagaagttttacatgcccaagaaggccacagaactgaaacatcttcagtgtctagaagaagaactcaaacctctggaggaagtgctaaatttagctcacagcaaaaactttcacttcgaagtcagggacgtagtcagcaatatcaacgtatttgttctggaactaaagggatctgaaacaacattcatgtgtgaatatgctgatgagacagcaaccattgtagaatttctgaacagatggattacctttagtcaaagcatcatctcaacactgacttga

SEQ ID NO: 188 - DNA, 399 bp, Artificial Sequence
  IL-2 analog 82
cctacttcaagttctacaaagaaaacacagctacaactggagcatttacgtctggatttagaaatgattttgaatggaattaataattacaagaatcccaaactcaccaggatgctcacatttaagttttacatgcccaagaaggccacagaactgaaacatcttcagtgtctagaagaagaactcaaacctctggaggaagtgctaaatttagctcaaagcaaaaactttcactttgaccccagggacgaagtgagcaatatcaacgtatttgttctggaactaaagggatctgaaacaacattcatgtgtgaatatgctgatgagacagcaaccattgtagaatttctgaacagatggattacctttagtcaaagcatcatctcaacactgacttga

SEQ ID NO: 189 - DNA, 399 bp, Artificial Sequence
  IL-2 analog 83
cctacttcaagttctacaaagaaaacacagctacaactggagcatttacgtcgtgatttagaaatgattttgaatggaattaataattacaagaatcccaaactcaccaggatgctcacatttaagttttacatgcccaagaaggccacagaactgaaacatcttcagtgtctagaagaagaactcaaacctctggaggaagtgctaaatttagctcaaagcaaaaactttcactttgaccccagggacgaagtgagcaatatcaacgtatttgttctggaactaaagggatctgaaacaacattcatgtgtgaatatgctgatgagacagcaaccattgtagaatttctgaacagatggattacctttagtcaaagcatcatctcaacactgacttga

SEQ ID NO: 190 - DNA, 399 bp, Artificial Sequence
  IL-2 analog 84
cctacttcaagttctacaaagaaaacacagctacaactggagcatttacgtctggatttagaaatgattttgaatggaattaataattacaagaatcccaaactcaccaggatgctcacatttaagttttacatgcccaagaaggccacagaactgaaacatcttcagtgtctagaagaagaactcaaacctctggaggaagtgctaaatttagctcaaagcaaaaactttcacgtggatcccagggacgaagtgagcaatatcaacgtatttgttctggaactaaagggatctgaaacaacattcatgtgtgaatatgctgatgagacagcaaccattgtagaatttctgaacagatggattacctttagtcaaagcatcatctcaacactgacttga

SEQ ID NO: 191 - DNA, 399 bp, Artificial Sequence
  IL-2 analog 85
cctacttcaagttctacaaagaaaacacagctacaactggagcatttactgctggatttacagatgattttgaatggaattaataattacaagaatcccaaactcaccaggatgctcacatttaagttttacatgcccaagaaggccacagaactgaaacatcttcagtgtctagaagaagaactcaaacctctggaggaagtgctaaatttagctcaaagcaaaaactttcacttcgaacccagggacgtagtcagcaatatcaacgtatttgttctggaactaaagggatctgaaacaacattcatgtgtgaatatgctgatgagacagcaaccattgtagaatttctgaacagatggattacctttagtcaaagcatcatctcaacactgacttga

SEQ ID NO: 192 - DNA, 399 bp, Artificial Sequence
  IL-2 analog 86
cctacttcaagttctacaaagaaaacacagctacaactggagcatttacgtctggatttagaaatgattttgaatggaattaataattacaagaatcccaaactcaccaggatgctcacatttaagttttacatgcccaagaaggccacagaactgaaacatcttcagtgtctagaagaagaactcaaacctctggaggaagtgctaaatttagctcaaagcaaaaactttcacttcgaacccagggacgtagtcagcaatatcaacgtatttgttctggaactaaagggatctgaaacaacattcatgtgtgaatatgctgatgagacagcaaccattgtagaatttctgaacagatggattacctttagtcaaagcatcatctcaacactgacttga

SEQ ID NO: 193 - DNA, 399 bp, Artificial Sequence
  IL-2 analog 87
cctacttcaagttctacaaagaaaacacagctacaactggagcatttacgtcgtgatttagaaatgattttgaatggaattaataattacaagaatcccaaactcaccaggatgctcacatttaagttttacatgcccaagaaggccacagaactgaaacatcttcagtgtctagaagaagaactcaaacctctggaggaagtgctaaatttagctcaaagcaaaaactttcacttcgaacccagggacgtagtcagcaatatcaacgtatttgttctggaactaaagggatctgaaacaacattcatgtgtgaatatgctgatgagacagcaaccattgtagaatttctgaacagatggattacctttagtcaaagcatcatctcaacactgacttga

SEQ ID NO: 194 - DNA, 399 bp, Artificial Sequence
  IL-2 analog 88
cctacttcaagttctacaaagaaaacacagctacaactggagcatttactgctggatttacagatgattttgaatggaattaataattacaagaatcccaaactcaccaggatgctcacatttaagttttacatgcccaagaaggccacagaactgaaacatcttcagtgtctagaagacgaactcaaacctctggaggaagtgctaaatttagctcaaagcaaaaactttcacttcgaacccagggacgtagtcagcaatatcaacgtatttgttctggaactaaagggatctgaaacaacattcatgtgtgaatatgctgatgagacagcaaccattgtagaatttctgaacagatggattacctttagtcaaagcatcatctcaacactgacttga

SEQ ID NO: 195 - DNA, 399 bp, Artificial Sequence
  IL-2 analog 89
cctacttcaagttctacaaagaaaacacagctacaactggagcatttactgctggatttacagatgattttgaatggaattaataattacaagaatcccaaactcaccgcgatgctcacatttaagttttacatgcccaagaaggccacagaactgaaacatcttcagtgtctagaagaagaactcaaacctctggagcaggtgctaaatttagctcaaagcaaaaactttcacttcgaacccagggacgtagtcagcaatatcaacgtatttgttctggaactaaagggatctgaaacaacattcatgtgtgaatatgctgatgagacagcaaccattgtagaatttctgaacagatggattacctttagtcaaagcatcatctcaacactgacttga

SEQ ID NO: 196 - DNA, 399 bp, Artificial Sequence
  IL-2 analog 90
cctacttcaagttctacaaagaaaacacagctacaactggagcatttactgctggatttacagatgattttgaatggaattaataattacaagaatcccaaactcaccaggatgctcacatggaagttttacatgcccaagaaggccacagaactgaaacatcttcagtgtctagaagaagaactcaaacctctggaggaagtgctaaatttagctcaaagcaaaaactttcacttcgaacccagggacgtagtcagcaatatcaacgtatttgttctggaactaaagggatctgaaacaacattcatgtgtgaatatgctgatgagacagcaaccattgtagaatttctgaacagatggattacctttagtcaaagcatcatctcaacactgacttga

SEQ ID NO: 197 - DNA, 399 bp, Artificial Sequence
  IL-2 analog 91
cctacttcaagttctacaaagaaaacacagctacaactggagcatttactgctggatttacagatgattttgaatggaattaataattacaagaatcccaaactcaccaggatgctcacatttaagttttacatgcccaagaaggccacagaactgaaacatcttcagtgtctagaacaagaactcaaacctctggaggaagtgctaaatttagctcaaagcaaaaactttcacttcgaacccagggacgtagtcagcaatatcaacgtatttgttctggaactaaagggatctgaaacaacattcatgtgtgaatatgctgatgagacagcaaccattgtagaatttctgaacagatggattacctttagtcaaagcatcatctcaacactgacttga

SEQ ID NO: 198 - DNA, 399 bp, Artificial Sequence
  IL-2 analog 92
cctacttcaagttctacaaagaaaacacagctacaactggagcatttactgctggatttacagatgattttgaatggaattaataattacaagaatcccaaactcaccaggatgctcacatttaagttttacatgcccaagaaggccacagaactgaaacatcttcagtgtctagaagaagaactcaaacctctggaggaagtgctaaatttagctcaaagcaaaaactttcacttcgaacccagggacgtagtcagcaatatcaacacatttgttctggaactaaagggatctgaaacaacattcatgtgtgaatatgctgatgagacagcaaccattgtagaatttctgaacagatggattacctttagtcaaagcatcatctcaacactgacttga

SEQ ID NO: 199 - DNA, 399 bp, Artificial Sequence
  IL-2 analog 93
cctacttcaagttctacaaagaaaacacagctacaactggagcatttactgctggatttacagatgattttgaatggaattaataattacaagaatcccaaactcaccaggatgctcacatttaagttttacatgcccaagaaggccacagaactgaaacatcttcagtgtctagaagaagaactcaaacctctggaggaagtgctaaatttagctcaaagcaaaaactttcacttcgaacccagggaggtagtcagcaatatcaacacatttgttctggaactaaagggatctgaaacaacattcatgtgtgaatatgctgatgagacagcaaccattgtagaatttctgaacagatggattacctttagtcaaagcatcatctcaacactgacttga

SEQ ID NO: 200 - DNA, 399 bp, Artificial Sequence
  IL-2 analog 94
cctacttcaagttctacaaagaaaacacagctacaactggagcatttactgctggatttacagatgattttgaatggaattaataattacaagaatcccaaactcaccaggatgctcacatttaagttttacatgcccaagaaggccacagaactgaaacatcttcagtgtctagaagaagaactcaaacctctggaggaagtgctaaatttagctcaaagcaaaaactttcacttcgaacccagggacgtagtcagcaatatcaacgtatttgttttcgaattcaagggatctgaaacaacattcatgtgtgaatatgctgatgagacagcaaccattgtagaatttctgaacagatggattacctttagtcaaagcatcatctcaacactgacttga

SEQ ID NO: 201 - DNA, 399 bp, Artificial Sequence
  IL-2 analog 95
cctacttcaagttctacaaagaaaacacagctacaactggagcatttactgctggatttacagatgattttgaatggaattaataattacaagaatcccaaactcaccaggatgctcacatttaagttttacatgcccaagaaggccacagaactgaaacatcttcagtgtctagaagaagaactcaaacctctggaggaagggctaaatttagctcaaagcaaaaactttcacttcgaacccagggacgtagtcagcaatatcaacgtatttgttctggaactaaagggatctgaaacaacattcatgtgtgaatatgctgatgagacagcaaccattgtagaatttctgaacagatggattacctttagtcaaagcatcatctcaacactgacttga

SEQ ID NO: 202 - DNA, 399 bp, Artificial Sequence
  IL-2 analog 96
cctacttcaagttctacaaagaaaacacagctacaactggagcatttactgctggatttacagatgattttgaatggaattaataattacaagaatcccaaactcaccaggatgctcacatttaagttttacatgcccaagaaggccacagaactgaaacatcttcagtgtctagaagaagaactcaaacctctggaggaagggctaaatttagctgcaagcaaaaactttcacttcgaacccagggacgtagtcagcaatatcaacgtatttgttctggaactaaagggatctgaaacaacattcatgtgtgaatatgctgatgagacagcaaccattgtagaatttctgaacagatggattacctttagtcaaagcatcatctcaacactgacttga

SEQ ID NO: 203 - DNA, 399 bp, Artificial Sequence
  IL-2 analog 97
cctacttcaagttctacaaagaaaacacagctacaactggagcatttactgctggatttacagatgattttgaatggaattaataattacaagaatcccaaactcaccgcgatgctcacatttaagttttacatgcccaagaaggccacagaactgaaacatcttcagtgtctagaagaagaactcaaacctctggaggaagtgctaaatttagctcaaagcaaaaactttcactttgaccccagggacttaatcagcaatatcaacgtatttgttctggaactaaagggatctgaaacaacattcatgtgtgaatatgctgatgagacagcaaccattgtagaatttctgaacagatggattacctttagtcaaagcatcatctcaacactgacttga

SEQ ID NO: 204 - DNA, 399 bp, Artificial Sequence
  IL-2 analog 98
cctacttcaagttctacaaagaaaacacagctacaactggagcatttactgctggatttacagatgattttgaatggaattaataattacaagaatcccaaactcaccgcgatgctcacatttaagttttacatgcccaagaaggccacagaactgaaacatcttcagtgtctagaagaagaactcaaacctctggaggaagtgctaaatttagctcaaagcaaaaactttcactttgagcccagggacgtaatcagcaatatcaacgtatttgttctggaactaaagggatctgaaacaacattcatgtgtgaatatgctgatgagacagcaaccattgtagaatttctgaacagatggattacctttagtcaaagcatcatctcaacactgacttga

SEQ ID NO: 205 - DNA, 399 bp, Artificial Sequence
  IL-2 analog 99
cctacttcaagttctacaaagaaaacacagctacaactggagcatttactgctggatttacagatgattttgaatggaattaataattacaagaatcccaaactcaccgcgatgctcacatttaagttttacatgcccaagaaggccacagaactgaaacatcttcagtgtctagaagaagaactcaaacctctggaggaagtgctaaatttagctcaaagcaaaaactttcactttgagcccagggacttagtcagcaatatcaacgtatttgttctggaactaaagggatctgaaacaacattcatgtgtgaatatgctgatgagacagcaaccattgtagaatttctgaacagatggattacctttagtcaaagcatcatctcaacactgacttga

SEQ ID NO: 206 - DNA, 399 bp, Artificial Sequence
  IL-2 analog 100
cctacttcaagttctacaaagaaaacacagctacaactggagcatttactgctggatttacagatgattttgaatggaattaataattacaagaatcccaaactcaccaggatgctcacatttaagttttacatgcccaagaaggccacagaactgaaacatcttcagtgtctagaagaagaactcaaacctctggaggaagtgctaaatttagctcaaagcaaaaactttcacttcgaacccagggactacgtcagcaatatcaacgtatttgttctggaactaaagggatctgaaacaacattcatgtgtgaatatgctgatgagacagcaaccattgtagaatttctgaacagatggattacctttagtcaaagcatcatctcaacactgacttga

SEQ ID NO: 207 - DNA, 399 bp, Artificial Sequence
  IL-2 analog 101
cctacttcaagttctacaaagaaaacacagctacaactggagcatttactgctggatttacagatgattttgaatggaattaataattacaagaatcccaaactcaccaggatgctcacatttaagttttacatgcccaagaaggccacagaactgaaacatcttcagtgtctagaagaagaactcaaacctctggaggaagtgctaaatttagctcaaagcaaaaactttcacttcgaacccagggacctggccagcaatatcaacgtatttgttctggaactaaagggatctgaaacaacattcatgtgtgaatatgctgatgagacagcaaccattgtagaatttctgaacagatggattacctttagtcaaagcatcatctcaacactgacttga

SEQ ID NO: 208 - DNA, 399 bp, Artificial Sequence
  IL-2 analog 102
cctacttcaagttctacaaagaaaacacagctacaactggagcatttactgctggatttacagatgattttgaatggaattaataattacaagaatcccaaactcaccaggatgctcacatttaagttttacatgcccaagaaggccacagaactgaaacatcttcagtgtctagaagaagaactcaaacctctggaggaagtgctaaatttagctcaaagcaaaaactttcacttcgaacccagggacgtagtcagcaatatcaacgtaattgttctggaactaaagggatctgaaacaacattcatgtgtgaatatgctgatgagacagcaaccattgtagaatttctgaacagatggattacctttagtcaaagcatcatctcaacactgacttga

SEQ ID NO: 209 - DNA, 399 bp, Artificial Sequence
  IL-2 analog 103
cctacttcaagttctacaaagaaaacacagctacaactggagcatttacgtctggatttagaaatgattttgaatggaattaataattacaagaatcccaaactcaccgcgatgctcacatttaagttttacatgcccaagaaggccacagaactgaaacatcttcagtgtctagaagaagaactcaaacctctggaggaagtgctaaatttagctcaaagcaaaaactttcacttcgaacccagggacgtagtcagcaatatcaacgtatttgttctggaactaaagggatctgaaacaacattcatgtgtgaatatgctgatgagacagcaaccattgtagaatttctgaacagatggattacctttagtcaaagcatcatctcaacactgacttga

SEQ ID NO: 210 - DNA, 399 bp, Artificial Sequence
  IL-2 analog 104
cctacttcaagttctacaaagaaaacacagctacaactggagcatttacgtctggatttagaaatgattttgaatggaattaataattacaagaatcccaaactcaccaggatgctcacatttaagttttacatgcccaagaaggccacagaactgaaacatcttcagtgtctagaagacgaactcaaacctctggaggaagtgctaaatttagctcaaagcaaaaactttcacttcgaacccagggacgtagtcagcaatatcaacgtatttgttctggaactaaagggatctgaaacaacattcatgtgtgaatatgctgatgagacagcaaccattgtagaatttctgaacagatggattacctttagtcaaagcatcatctcaacactgacttga

SEQ ID NO: 211 - DNA, 399 bp, Artificial Sequence
  IL-2 analog 105
cctacttcaagttctacaaagaaaacacagctacaactggagcatttacgtctggatttagaaatgattttgaatggaattaataattacaagaatcccaaactcaccaggatgctcacatttaagttttacatgcccaagaaggccacagaactgaaacatcttcagtgtctagaagaagaactcaaacctctggaggacgtgctaaatttagctcaaagcaaaaactttcacttcgaacccagggacgtagtcagcaatatcaacgtatttgttctggaactaaagggatctgaaacaacattcatgtgtgaatatgctgatgagacagcaaccattgtagaatttctgaacagatggattacctttagtcaaagcatcatctcaacactgacttga

SEQ ID NO: 212 - protein, 133 aa, Artificial Sequence
  General Formula 1
  MISC_FEATURE (1): Xaa is a deletion
  MISC_FEATURE (18): Xaa is leucine (L) or arginine (R)
  MISC_FEATURE (19): Xaa is leucine (L) or tyrosine (Y)
  MISC_FEATURE (22): Xaa is glutamic acid (E) or glutamine (Q)
  MISC_FEATURE (38): Xaa is alanine (A), aspartic acid (D), or arginine (R)
  MISC_FEATURE (42): Xaa is alanine (A), phenylalanine (F), lysine (K), or tryptophan (W)
  MISC_FEATURE (43): Xaa is glutamic acid (E), lysine (K), or glutamine (Q)
  MISC_FEATURE (45): Xaa is alanine (A) or tyrosine (Y)
  MISC_FEATURE (61): Xaa is aspartic acid (D), glutamic acid (E), glutamine (Q), or arginine (R)
  MISC_FEATURE (68): Xaa is aspartic acid (D) or glutamic acid (E)
  MISC_FEATURE (74): Xaa is histidine (H) or glutamine (Q)
  MISC_FEATURE (80): Xaa is phenylalanine (F), leucine (L), valine (V), or tyrosine (Y)
  MISC_FEATURE (81): Xaa is aspartic acid (D), glutamic acid (E), or arginine (R)
  MISC_FEATURE (84): Xaa is aspartic acid (D) or glutamic acid (E)
  MISC_FEATURE (85): Xaa is alanine (A), glutamic acid (E), glycine (G), leucine (L), valine (V), tryptophan (W), or tyrosine (Y)
  MISC_FEATURE (86): Xaa is alanine (A), glycine (G), isoleucine (I), or valine (V)
  MISC_FEATURE (91): Xaa is threonine (T) or valine (V)
  MISC_FEATURE (92): Xaa is phenylalanine (F), isoleucine (I), or tyrosine (Y)
  MISC_FEATURE (94): Xaa is phenylalanine (F) or leucine (L)
  MISC_FEATURE (96): Xaa is phenylalanine (F) or leucine (L)
XPTSSSTKKTQLQLEHLXXDLXMILNGINNYKNPKLTXMLTXXFXMPKKATELKHLQCLEXELKPLEXVLNLAXSKNFHXXPRXXXSNINXXVXEXKGSETTFMCEYADETATIVEFLNRWITFSQSIISTLT

SEQ ID NO: 213 - protein, 133 aa, Artificial Sequence
  General Formula 2
  MISC_FEATURE (1): Xaa is a deletion
  MISC_FEATURE (18): Xaa is leucine (L) or arginine (R)
  MISC_FEATURE (22): Xaa is glutamic acid (E) or glutamine (Q)
  MISC_FEATURE (38): Xaa is alanine (A) or arginine (R)
  MISC_FEATURE (42): Xaa is phenylalanine (F) or lysine (K)
  MISC_FEATURE (61): Xaa is aspartic acid (D) or glutamic acid (E)
  MISC_FEATURE (68): Xaa is aspartic acid (D) or glutamic acid (E)
  MISC_FEATURE (81): Xaais aspartic acid (D) or glutamic acid (E)
  MISC_FEATURE (85): Xaa is leucine (L) or valine (V)
  MISC_FEATURE (86): Xaa is isoleucine (I) or valine (V)
XPTSSSTKKTQLQLEHLXLDLXMILNGINNYKNPKLTXMLTXKFYMPKKATELKHLQCLEXELKPLEXVLNLAQSKNFHFXPRDXXSNINVFVLELKGSETTFMCEYADETATIVEFLNRWITFSQSIISTLT

SEQ ID NO: 214 - DNA, 33 bp, Artificial Sequence
  primer #1 (IL2_L12F_F)
caaagaaaacacagtttcaactggagcatttac

SEQ ID NO: 215 - DNA, 33 bp, Artificial Sequence
  primer #2 (IL2_L12F_R)
gtaaatgctccagttgaaactgtgttttctttg

SEQ ID NO: 216 - DNA, 33 bp, Artificial Sequence
  primer #3 (IL2_L12V_F)
caaagaaaacacaggtacaactggagcatttac

SEQ ID NO: 217 - DNA, 33 bp, Artificial Sequence
  primer #4 (IL2_L12V_R)
gtaaatgctccagttgtacctgtgttttctttg

SEQ ID NO: 218 - DNA, 39 bp, Artificial Sequence
  primer #5 (IL2_L18R_L19R_Q22E_F)
ctggagcatttacgtcgtgatttagaaatgattttgaat

SEQ ID NO: 219 - DNA, 39 bp, Artificial Sequence
  primer #6 (IL2_L18R_L19R_Q22E_R)
attcaaaatcatttctaaatcacgacgtaaatgctccag

SEQ ID NO: 220 - DNA, 39 bp, Artificial Sequence
  primer #7 (IL2_L18R_Q22E_F)
ctggagcatttacgtctggatttagaaatgattttgaat

SEQ ID NO: 221 - DNA, 39 bp, Artificial Sequence
  primer #8 (IL2_L18R_Q22E_R)
attcaaaatcatttctaaatccagacgtaaatgctccag

SEQ ID NO: 222 - DNA, 33 bp, Artificial Sequence
  primer #9 (IL2_L19F_F)
gagcatttactgttcgatttacagatgattttg

SEQ ID NO: 223 - DNA, 33 bp, Artificial Sequence
  primer #10 (IL2_L19F_R)
caaaatcatctgtaaatcgaacagtaaatgctc

SEQ ID NO: 224 - DNA, 33 bp, Artificial Sequence
  primer #11 (IL2_L19V_F)
gagcatttactggtggatttacagatgattttg

SEQ ID NO: 225 - DNA, 33 bp, Artificial Sequence
  primer #12 (IL2_L19V_R)
caaaatcatctgtaaatccaccagtaaatgctc

SEQ ID NO: 226 - DNA, 33 bp, Artificial Sequence
  primer #13 (IL2_L19Y_F)
caactggagcatttactgtacgatttacagatg

SEQ ID NO: 227 - DNA, 33 bp, Artificial Sequence
  primer #14 (IL2_L19Y_R)
catctgtaaatcgtacagtaaatgctccagttg

SEQ ID NO: 228 - DNA, 34 bp, Artificial Sequence
  primer #15 (IL2_D20F_F)
ggagcatttactgctgtttttacagatgattttg

SEQ ID NO: 229 - DNA, 34 bp, Artificial Sequence
  primer #16 (IL2_D20F_R)
caaaatcatctgtaaaaacagcagtaaatgctcc

SEQ ID NO: 230 - DNA, 33 bp, Artificial Sequence
  primer #17 (IL2_D20V_F)
gagcatttactgctggttttacagatgattttg

SEQ ID NO: 231 - DNA, 33 bp, Artificial Sequence
  primer #18 (IL2_D20V_R)
caaaatcatctgtaaaaccagcagtaaatgctc

SEQ ID NO: 232 - DNA, 33 bp, Artificial Sequence
  primer #19 (IL2_K32C_F)
ggaattaataattactgtaatcccaaactcacc

SEQ ID NO: 233 - DNA, 33 bp, Artificial Sequence
  primer #20 (IL2_K32C_R)
ggtgagtttgggattacagtaattattaattcc

SEQ ID NO: 234 - DNA, 33 bp, Artificial Sequence
  primer #21 (IL2_K35C_F)
aattacaagaatccctgtctcaccaggatgctc

SEQ ID NO: 235 - DNA, 33 bp, Artificial Sequence
  primer #22 (IL2_K35C_R)
gagcatcctggtgagacagggattcttgtaatt

SEQ ID NO: 236 - DNA, 33 bp, Artificial Sequence
  primer #23 (IL2_K35E_F)
taattacaagaatcccgaactcaccgcgatgct

SEQ ID NO: 237 - DNA, 33 bp, Artificial Sequence
  primer #24 (IL2_K35E_R)
agcatcgcggtgagttcgggattcttgtaatta

SEQ ID NO: 238 - DNA, 25 bp, Artificial Sequence
  primer #25 (IL2_R38A_F)
ccaaactcaccgcgatgctcacatt

SEQ ID NO: 239 - DNA, 25 bp, Artificial Sequence
  primer #26 (IL2_R38A_R)
aatgtgagcatcgcggtgagtttgg

SEQ ID NO: 240 - DNA, 33 bp, Artificial Sequence
  primer #27 (IL2_R38A_F42F_F)
caccgcgatgctcacatttaagttttacatgcc

SEQ ID NO: 241 - DNA, 33 bp, Artificial Sequence
  primer #28 (IL2_R38A_F42F_R)
ggcatgtaaaacttaaatgtgagcatcgcggtg

SEQ ID NO: 242 - DNA, 25 bp, Artificial Sequence
  primer #29 (IL2_A38R_F)
ccaaactcaccaggatgctcacatt

SEQ ID NO: 243 - DNA, 25 bp, Artificial Sequence
  primer #30 (IL2_A38R_R)
aatgtgagcatcctggtgagtttgg

SEQ ID NO: 244 - DNA, 30 bp, Artificial Sequence
  primer #31 (IL2_R38D_F)
aagaatcccaaactcaccgatatgctcaca

SEQ ID NO: 245 - DNA, 30 bp, Artificial Sequence
  primer #32 (IL2_R38D_R)
tgtgagcatatcggtgagtttgggattctt

SEQ ID NO: 246 - DNA, 30 bp, Artificial Sequence
  primer #33 (IL2_F42A_F)
ccaggatgctcacagctaagttttacatgc

SEQ ID NO: 247 - DNA, 30 bp, Artificial Sequence
  primer #34 (IL2_F42A_R)
gcatgtaaaacttagctgtgagcatcctgg

SEQ ID NO: 248 - DNA, 30 bp, Artificial Sequence
  primer #35 (IL2_F42K_F)
ccaggatgctcacaaagaagttttacatgc

SEQ ID NO: 249 - DNA, 30 bp, Artificial Sequence
  primer #36 (IL2_F42K_R)
gcatgtaaaacttctttgtgagcatcctgg

SEQ ID NO: 250 - DNA, 30 bp, Artificial Sequence
  primer #37 (IL2_F42K_K43E_F)
atgctcacaaaggagttttacatgcccaag

SEQ ID NO: 251 - DNA, 30 bp, Artificial Sequence
  primer #38 (IL2_F42K_K43E_R)
cttgggcatgtaaaactcctttgtgagcat

SEQ ID NO: 252 - DNA, 30 bp, Artificial Sequence
  primer #39 (IL2_F42K_K43Q_F)
atgctcacaaagcagttttacatgcccaag

SEQ ID NO: 253 - DNA, 30 bp, Artificial Sequence
  primer #40 (IL2_F42K_K43Q_R)
cttgggcatgtaaaactgctttgtgagcat

SEQ ID NO: 254 - DNA, 30 bp, Artificial Sequence
  primer #41 (IL2_K42F_F)
ccaggatgctcacatttaagttttacatgc

SEQ ID NO: 255 - DNA, 30 bp, Artificial Sequence
  primer #42 (IL2_K42F_R)
gcatgtaaaacttaaatgtgagcatcctgg

SEQ ID NO: 256 - DNA, 39 bp, Artificial Sequence
  primer #43 (IL2_K42F_F_long)
ctcaccaggatgctcacatttaagttttacatgcccaag

SEQ ID NO: 257 - DNA, 39 bp, Artificial Sequence
  primer #44 (IL2_K42F_R_long)
cttgggcatgtaaaacttaaatgtgagcatcctggtgag

SEQ ID NO: 258 - DNA, 33 bp, Artificial Sequence
  primer #45 (IL2_F42W_F)
accaggatgctcacatggaagttttacatgccc

SEQ ID NO: 259 - DNA, 33 bp, Artificial Sequence
  primer #46 (IL2_F42W_R)
gggcatgtaaaacttccatgtgagcatcctggt

SEQ ID NO: 260 - DNA, 33 bp, Artificial Sequence
  primer #47 (IL2_K43C_F)
aggatgctcacattttgtttttacatgcccaag

SEQ ID NO: 261 - DNA, 33 bp, Artificial Sequence
  primer #48 (IL2_K43C_R)
cttgggcatgtaaaaacaaaatgtgagcatcct

SEQ ID NO: 262 - DNA, 19 bp, Artificial Sequence
  primer #49 (IL2_Y45A_F)
gaagtttgccatgcccaag

SEQ ID NO: 263 - DNA, 19 bp, Artificial Sequence
  primer #50 (IL2_Y45A_R)
cttgggcatggcaaacttc

SEQ ID NO: 264 - DNA, 34 bp, Artificial Sequence
  primer #51 (IL2_Y45A_F_long)
gctcacaaagaagtttgccatgcccaagaaggcc

SEQ ID NO: 265 - DNA, 34 bp, Artificial Sequence
  primer #52 (IL2_Y45A_R_long)
ggccttcttgggcatggcaaacttctttgtgagc

SEQ ID NO: 266 - DNA, 33 bp, Artificial Sequence
  primer #53 (IL2_K48C_F)
aagttttacatgccctgtaaggccacagaactg

SEQ ID NO: 267 - DNA, 33 bp, Artificial Sequence
  primer #54 (IL2_K48C_R)
cagttctgtggccttacagggcatgtaaaactt

SEQ ID NO: 268 - DNA, 33 bp, Artificial Sequence
  primer #55 (IL2_K49C_F)
ttttacatgcccaagtgtgccacagaactgaaa

SEQ ID NO: 269 - DNA, 33 bp, Artificial Sequence
  primer #56 (IL2_K49C_R)
tttcagttctgtggcacacttgggcatgtaaaa

SEQ ID NO: 270 - DNA, 33 bp, Artificial Sequence
  primer #57 (IL2_E61D_F)
cttcagtgtctagaagacgaactcaaacctctg

SEQ ID NO: 271 - DNA, 33 bp, Artificial Sequence
  primer #58 (IL2_E61D_R)
cagaggtttgagttcgtcttctagacactgaag

SEQ ID NO: 272 - DNA, 33 bp, Artificial Sequence
  primer #59 (IL2_E61Q_F)
cttcagtgtctagaacaagaactcaaacctctg

SEQ ID NO: 273 - DNA, 33 bp, Artificial Sequence
  primer #60 (IL2_E61Q_R)
cagaggtttgagttcttgttctagacactgaag

SEQ ID NO: 274 - DNA, 30 bp, Artificial Sequence
  primer #61 (IL2_E61R_F)
cttcagtgtctagaacgggaactcaaacct

SEQ ID NO: 275 - DNA, 30 bp, Artificial Sequence
  primer #62 (IL2_E61R_R)
aggtttgagttcccgttctagacactgaag

SEQ ID NO: 276 - DNA, 33 bp, Artificial Sequence
  primer #63 (IL2_E68D_F)
ctcaaacctctggaggacgtgctaaatttagct

SEQ ID NO: 277 - DNA, 33 bp, Artificial Sequence
  primer #64 (IL2_E68D_R)
agctaaatttagcacgtcctccagaggtttgag

SEQ ID NO: 278 - DNA, 33 bp, Artificial Sequence
  primer #65 (IL2_E68Q_F)
ctcaaacctctggagcaggtgctaaatttagct

SEQ ID NO: 279 - DNA, 33 bp, Artificial Sequence
  primer #66 (IL2_E68Q_R)
agctaaatttagcacctgctccagaggtttgag

SEQ ID NO: 280 - DNA, 32 bp, Artificial Sequence
  primer #67 (IL2_V69G_F)
caaacctctggaggaagggctaaatttagctc

SEQ ID NO: 281 - DNA, 32 bp, Artificial Sequence
  primer #68 (IL2_V69G_R)
gagctaaatttagcccttcctccagaggtttg

SEQ ID NO: 282 - DNA, 40 bp, Artificial Sequence
  primer #69 (IL2_V69G_Q74A_F)
ctggaggaagggctaaatttagctgcaagcaaaaactttc

SEQ ID NO: 283 - DNA, 40 bp, Artificial Sequence
  primer #70 (IL2_V69G_Q74A_R)
gaaagtttttgcttgcagctaaatttagcccttcctccag

SEQ ID NO: 284 - DNA, 24 bp, Artificial Sequence
  primer #71 (IL2_Q74H_F)
ctaaatttagctcacagcaaaaac

SEQ ID NO: 285 - DNA, 24 bp, Artificial Sequence
  primer #72 (IL2_Q74H_R)
gtttttgctgtgagctaaatttag

SEQ ID NO: 286 - DNA, 33 bp, Artificial Sequence
  primer #73 (IL2_K76C_F)
aatttagctcaaagctgtaactttcacttaaga

SEQ ID NO: 287 - DNA, 33 bp, Artificial Sequence
  primer #74 (IL2_K76C_R)
tcttaagtgaaagttacagctttgagctaaatt

SEQ ID NO: 288 - DNA, 32 bp, Artificial Sequence
  primer #75 (IL2_L80D_R81E_F)
aaagcaaaaactttcacgacgaacccagggac

SEQ ID NO: 289 - DNA, 32 bp, Artificial Sequence
  primer #76 (IL2_L80D_R81E_R)
gtccctgggttcgtcgtgaaagtttttgcttt

SEQ ID NO: 290 - DNA, 29 bp, Artificial Sequence
  primer #77 (IL2_L80F_F)
gcaaaaactttcactttagacccagggac

SEQ ID NO: 291 - DNA, 29 bp, Artificial Sequence
  primer #78 (IL2_L80F_R)
gtccctgggtctaaagtgaaagtttttgc

SEQ ID NO: 292 - DNA, 29 bp, Artificial Sequence
  primer #79 (IL2_L80F_R81D_F)
gcaaaaactttcactttgaccccagggac

SEQ ID NO: 293 - DNA, 29 bp, Artificial Sequence
  primer #80 (IL2_L80F_R81D_R)
gtccctggggtcaaagtgaaagtttttgc

SEQ ID NO: 294 - DNA, 32 bp, Artificial Sequence
  primer #81 (IL2_L80F_R81E_F)
aaagcaaaaactttcacttcgaacccagggac

SEQ ID NO: 295 - DNA, 32 bp, Artificial Sequence
  primer #82 (IL2_L80F_R81E_R)
gtccctgggttcgaagtgaaagtttttgcttt

SEQ ID NO: 296 - DNA, 32 bp, Artificial Sequence
  primer #83 (IL2_L80V_R81D_F)
aaagcaaaaactttcacgtggatcccagggac

SEQ ID NO: 297 - DNA, 32 bp, Artificial Sequence
  primer #84 (IL2_L80V_R81D_R)
gtccctgggatccacgtgaaagtttttgcttt

SEQ ID NO: 298 - DNA, 32 bp, Artificial Sequence
  primer #85 (IL2_L80W_R81E_F)
aaagcaaaaactttcactgggaacccagggac

SEQ ID NO: 299 - DNA, 32 bp, Artificial Sequence
  primer #86 (IL2_L80W_R81E_R)
gtccctgggttcccagtgaaagtttttgcttt

SEQ ID NO: 300 - DNA, 29 bp, Artificial Sequence
  primer #87 (IL2_L80Y_R81D_F)
gcaaaaactttcactatgaccccagggac

SEQ ID NO: 301 - DNA, 29 bp, Artificial Sequence
  primer #88 (IL2_L80Y_R81D_R)
gtccctggggtcatagtgaaagtttttgc

SEQ ID NO: 302 - DNA, 32 bp, Artificial Sequence
  primer #89 (IL2_L80Y_R81E_F)
aaagcaaaaactttcactacgaacccagggac

SEQ ID NO: 303 - DNA, 32 bp, Artificial Sequence
  primer #90 (IL2_L80Y_R81E_R)
gtccctgggttcgtagtgaaagtttttgcttt

SEQ ID NO: 304 - DNA, 32 bp, Artificial Sequence
  primer #91 (IL2_L80Y_R81N_F)
aaagcaaaaactttcactacaaccccagggac

SEQ ID NO: 305 - DNA, 32 bp, Artificial Sequence
  primer #92 (IL2_L80Y_R81N_R)
gtccctggggttgtagtgaaagtttttgcttt

SEQ ID NO: 306 - DNA, 29 bp, Artificial Sequence
  primer #93 (IL2_L80Y_R81R_F)
gcaaaaactttcactatagacccagggac

SEQ ID NO: 307 - DNA, 29 bp, Artificial Sequence
  primer #94 (IL2_L80Y_R81R_R)
gtccctgggtctatagtgaaagtttttgc

SEQ ID NO: 308 - DNA, 31 bp, Artificial Sequence
  primer #95 (IL2_R81D_D84E_F)
ctttcacttagaccccagggagttaatcagc

SEQ ID NO: 309 - DNA, 31 bp, Artificial Sequence
  primer #96 (IL2_R81D_D84E_R)
gctgattaactccctggggtctaagtgaaag

SEQ ID NO: 310 - DNA, 34 bp, Artificial Sequence
  primer #97 (IL2_R81D_F)
caaaaactttcacttagaccccagggacttaatc

SEQ ID NO: 311 - DNA, 34 bp, Artificial Sequence
  primer #98 (IL2_R81D_R)
gattaagtccctggggtctaagtgaaagtttttg

SEQ ID NO: 312 - DNA, 51 bp, Artificial Sequence
  primer #99 (IL2_R81D_F_long)
ctcaaagcaaaaactttcacttagaccccagggacttaatcagcaaatatc

SEQ ID NO: 313 - DNA, 51 bp, Artificial Sequence
  primer #100 (IL2_R81D_R_long)
gatatttgctgattaagtccctggggtctaagtgaaagtttttgctttgag

SEQ ID NO: 314 - DNA, 43 bp, Artificial Sequence
  primer #101 (IL2_R81E_D84E_L85V_I86V_V91T_I92F_F)
gaacccagggaggtagtcagcaatatcaacacatttgttctgg

SEQ ID NO: 315 - DNA, 43 bp, Artificial Sequence
  primer #102 (IL2_R81E_D84E_L85V_I86V_V91T_I92F_R)
ccagaacaaatgtgttgatattgctgactacctccctgggttc

SEQ ID NO: 316 - DNA, 31 bp, Artificial Sequence
  primer #103 (IL2_R81E_F)
aaactttcacttagaacccagggacttaatc

SEQ ID NO: 317 - DNA, 31 bp, Artificial Sequence
  primer #104 (IL2_R81E_R)
gattaagtccctgggttctaagtgaaagttt

SEQ ID NO: 318 - DNA, 33 bp, Artificial Sequence
  primer #105 (IL2_P82G_F)
aactttcacttcgaaggcagggacgtagtcagc

SEQ ID NO: 319 - DNA, 33 bp, Artificial Sequence
  primer #106 (IL2_P82G_R)
gctgactacgtccctgccttcgaagtgaaagtt

SEQ ID NO: 320 - DNA, 33 bp, Artificial Sequence
  primer #107 (IL2_P82V_F)
aactttcacttcgaagtcagggacgtagtcagc

SEQ ID NO: 321 - DNA, 33 bp, Artificial Sequence
  primer #108 (IL2_P82V_R)
gctgactacgtccctgacttcgaagtgaaagtt

SEQ ID NO: 322 - DNA, 34 bp, Artificial Sequence
  primer #109 (IL2_D84E_F)
cttaagacccagggagttaatcagcaatatcaac

SEQ ID NO: 323 - DNA, 34 bp, Artificial Sequence
  primer #110 (IL2_D84E_R)
gttgatattgctgattaactccctgggtcttaag

SEQ ID NO: 324 - DNA, 32 bp, Artificial Sequence
  primer #111 (IL2_D84F_F)
cacttagaccccaggttcttaatcagcaatat

SEQ ID NO: 325 - DNA, 32 bp, Artificial Sequence
  primer #112 (IL2_D84F_R)
atattgctgattaagaacctggggtctaagtg

SEQ ID NO: 326 - DNA, 31 bp, Artificial Sequence
  primer #113 (IL2_D84V_F)
acttagaccccagggtcttaatcagcaatat

SEQ ID NO: 327 - DNA, 31 bp, Artificial Sequence
  primer #114 (IL2_D84V_R)
atattgctgattaagaccctggggtctaagt

SEQ ID NO: 328 - DNA, 35 bp, Artificial Sequence
  primer #115 (IL2_L85A_I86A_F)
ctttgaccccagggacgctgccagcaatatcaacg

SEQ ID NO: 329 - DNA, 35 bp, Artificial Sequence
  primer #116 (IL2_L85A_I86A_R)
cgttgatattgctggcagcgtccctggggtcaaag

SEQ ID NO: 330 - DNA, 30 bp, Artificial Sequence
  primer #117 (IL2_L85E_I86V_F)
cccagggacgaagtgagcaatatcaacgta

SEQ ID NO: 331 - DNA, 30 bp, Artificial Sequence
  primer #118 (IL2_L85E_I86V_R)
tacgttgatattgctcacttcgtccctggg

SEQ ID NO: 332 - DNA, 27 bp, Artificial Sequence
  primer #119 (IL2_L85F_I86L_F)
cccagggacttcctcagcaatatcaac

SEQ ID NO: 333 - DNA, 27 bp, Artificial Sequence
  primer #120 (IL2_L85F_I86L_R)
gttgatattgctgaggaagtccctggg

SEQ ID NO: 334 - DNA, 27 bp, Artificial Sequence
  primer #121 (IL2_L85F_I86V_F)
cccagggacttcgtcagcaatatcaac

SEQ ID NO: 335 - DNA, 27 bp, Artificial Sequence
  primer #122 (IL2_L85F_I86V_R)
gttgatattgctgacgaagtccctggg

SEQ ID NO: 336 - DNA, 27 bp, Artificial Sequence
  primer #123 (IL2_L85G_I86A_F)
cccagggacggagccagcaatatcaac

SEQ ID NO: 337 - DNA, 27 bp, Artificial Sequence
  primer #124 (IL2_L85G_I86A_R)
gttgatattgctggctccgtccctggg

SEQ ID NO: 338 - DNA, 35 bp, Artificial Sequence
  primer #125 (IL2_L85G_I86V_F)
ctttgaccccagggacggtgttagcaatatcaacg

SEQ ID NO: 339 - DNA, 35 bp, Artificial Sequence
  primer #126 (IL2_L85G_I86V_R)
cgttgatattgctaacccagtccctggggtcaaag

SEQ ID NO: 340 - DNA, 27 bp, Artificial Sequence
  primer #127 (IL2_L85I_I86V_F)
cccagggacatagtcagcaatatcaac

SEQ ID NO: 341 - DNA, 27 bp, Artificial Sequence
  primer #128 (IL2_L85I_I86V_R)
gttgatattgctgactatgtccctggg

SEQ ID NO: 342 - DNA, 34 bp, Artificial Sequence
  primer #129 (IL2_L85L_I86A_F)
cttcgaacccagggacctggccagcaatatcaac

SEQ ID NO: 343 - DNA, 34 bp, Artificial Sequence
  primer #130 (IL2_L85L_I86A_R)
gttgatattgctggccaggtccctgggttcgaag

SEQ ID NO: 344 - DNA, 34 bp, Artificial Sequence
  primer #131 (IL2_L85L_I86V_F)
ctttgagcccagggacttagtcagcaatatcaac

SEQ ID NO: 345 - DNA, 34 bp, Artificial Sequence
  primer #132 (IL2_L85L_I86V_R)
gttgatattgctgactaagtccctgggctcaaag

SEQ ID NO: 346 - DNA, 27 bp, Artificial Sequence
  primer #133 (IL2_L85T_I86G_F)
cccagggacacaggcagcaatatcaac

SEQ ID NO: 347 - DNA, 27 bp, Artificial Sequence
  primer #134 (IL2_L85T_I86G_R)
gttgatattgctgcctgtgtccctggg

SEQ ID NO: 348 - DNA, 29 bp, Artificial Sequence
  primer #135 (IL2_L85V_I86G_F)
cccagggacgtaggcagcaatatcaacgt

SEQ ID NO: 349 - DNA, 29 bp, Artificial Sequence
  primer #136 (IL2_L85V_I86G_R)
acgttgatattgctgcctacgtccctggg

SEQ ID NO: 350 - DNA, 31 bp, Artificial Sequence
  primer #137 (IL2_L85V_I86I_codon_F)
gaacccagggacgtaatcagcaatatcaacg

SEQ ID NO: 351 - DNA, 31 bp, Artificial Sequence
  primer #138 (IL2_L85V_I86I_codon_R)
cgttgatattgctgattacgtccctgggttc

SEQ ID NO: 352 - DNA, 30 bp, Artificial Sequence
  primer #139 (IL2_L85V_I86V_F)
gacccagggacgtagtcagcaatatcaacg

SEQ ID NO: 353 - DNA, 30 bp, Artificial Sequence
  primer #140 (IL2_L85V_I86V_R)
cgttgatattgctgactacgtccctgggtc

SEQ ID NO: 354 - DNA, 29 bp, Artificial Sequence
  primer #141 (IL2_L85W_I86V_F)
cccagggactgggtcagcaatatcaacgt

SEQ ID NO: 355 - DNA, 29 bp, Artificial Sequence
  primer #142 (IL2_L85W_I86V_R)
acgttgatattgctgacccagtccctggg

SEQ ID NO: 356 - DNA, 30 bp, Artificial Sequence
  primer #143 (IL2_L85W_I86V_Long_F)
tttgaccccagggactgggtcagcaatatc

SEQ ID NO: 357 - DNA, 30 bp, Artificial Sequence
  primer #144 (IL2_L85W_I86V_Long_R)
gatattgctgacccagtccctggggtcaaa

SEQ ID NO: 358 - DNA, 34 bp, Artificial Sequence
  primer #145 (IL2_L85Y_I86V_F)
cttcgaacccagggactacgtcagcaatatcaac

SEQ ID NO: 359 - DNA, 34 bp, Artificial Sequence
  primer #146 (IL2_L85Y_I86V_R)
gttgatattgctgacgtagtccctgggttcgaag

SEQ ID NO: 360 - DNA, 31 bp, Artificial Sequence
  primer #147 (IL2_I86V_V91T_I92F_F)
gtcagcaatatcaacacatttgttctggaac

SEQ ID NO: 361 - DNA, 31 bp, Artificial Sequence
  primer #148 (IL2_I86V_V91T_I92F_R)
gttccagaacaaatgtgttgatattgctgac

SEQ ID NO: 362 - DNA, 33 bp, Artificial Sequence
  primer #149 (IL2_S87C_F)
cccagggacttaatctgcaatatcaacgtaata

SEQ ID NO: 363 - DNA, 33 bp, Artificial Sequence
  primer #150 (IL2_S87C_R)
tattacgttgatattgcagattaagtccctggg

SEQ ID NO: 364 - DNA, 34 bp, Artificial Sequence
  primer #151 (IL2_N88F_F)
cagggacttaatcagctttatcaacgtatttgtt

SEQ ID NO: 365 - DNA, 34 bp, Artificial Sequence
  primer #152 (IL2_N88F_R)
aacaaatacgttgataaagctgattaagtccctg

SEQ ID NO: 366 - DNA, 33 bp, Artificial Sequence
  primer #153 (IL2_N88Q_F)
gggacttaatcagccaaatcaacgtaatagttc

SEQ ID NO: 367 - DNA, 33 bp, Artificial Sequence
  primer #154 (IL2_N88Q_R)
gaactattacgttgatttggctgattaagtccc

SEQ ID NO: 368 - DNA, 34 bp, Artificial Sequence
  primer #155 (IL2_N88V_F)
cagggacttaatcagcgttatcaacgtatttgtt

SEQ ID NO: 369 - DNA, 34 bp, Artificial Sequence
  primer #156 (IL2_N88V_R)
aacaaatacgttgataacgctgattaagtccctg

SEQ ID NO: 370 - DNA, 33 bp, Artificial Sequence
  primer #157 (IL2_I89F_F)
gacttaatcagcaatttcaacgtaatagttctg

SEQ ID NO: 371 - DNA, 33 bp, Artificial Sequence
  primer #158 (IL2_I89F_R)
cagaactattacgttgaaattgctgattaagtc

SEQ ID NO: 372 - DNA, 33 bp, Artificial Sequence
  primer #159 (IL2_V91E_I92F_F)
agcaatatcaacgaattcgttctggaactaaag

SEQ ID NO: 373 - DNA, 33 bp, Artificial Sequence
  primer #160 (IL2_V91E_I92F_R)
ctttagttccagaacgaattcgttgatattgct

SEQ ID NO: 374 - DNA, 33 bp, Artificial Sequence
  primer #161 (IL2_V91E_I92W_F)
agcaatatcaacgaatgggttctggaactaaag

SEQ ID NO: 375 - DNA, 33 bp, Artificial Sequence
  primer #162 (IL2_V91E_I92W_R)
ctttagttccagaacccattcgttgatattgct

SEQ ID NO: 376 - DNA, 34 bp, Artificial Sequence
  primer #163 (IL2_V91F_F)
cagcaatatcaactttatagttctggaactaaag

SEQ ID NO: 377 - DNA, 34 bp, Artificial Sequence
  primer #164 (IL2_V91F_R)
ctttagttccagaactataaagttgatattgctg

SEQ ID NO: 378 - DNA, 34 bp, Artificial Sequence
  primer #165 (IL2_V91T_F)
cagcaatatcaacacaatagttctggaactaaag

SEQ ID NO: 379 - DNA, 34 bp, Artificial Sequence
  primer #166 (IL2_V91T_R)
ctttagttccagaactattgtgttgatattgctg

SEQ ID NO: 380 - DNA, 32 bp, Artificial Sequence
  primer #167 (IL2_I92F_F)
gcaatatcaacgtatttgttctggaactaaag

SEQ ID NO: 381 - DNA, 32 bp, Artificial Sequence
  primer #168 (IL2_I92F_R)
ctttagttccagaacaaatacgttgatattgc

SEQ ID NO: 382 - DNA, 49 bp, Artificial Sequence
  primer #169 (IL2_I92F_F_long)
gacttaatcagcaatatcaacgtatttgttctggaactaaagggatctg

SEQ ID NO: 383 - DNA, 49 bp, Artificial Sequence
  primer #170 (IL2_I92F_R_long)
cagatccctttagttccagaacaaatacgttgatattgctgattaagtc

SEQ ID NO: 384 - DNA, 45 bp, Artificial Sequence
  primer #171 (IL2_I92F_F_long2)
cttaatcagcaatatcaacgtatttgttctggaactaaagggatc

SEQ ID NO: 385 - DNA, 45 bp, Artificial Sequence
  primer #172 (IL2_I92F_R_long2)
gatccctttagttccagaacaaatacgttgatattgctgattaag

SEQ ID NO: 386 - DNA, 32 bp, Artificial Sequence
  primer #173 (IL2_I92F_L94F_L96F_F)
caacgtatttgttttcgaattcaagggatctg

SEQ ID NO: 387 - DNA, 32 bp, Artificial Sequence
  primer #174 (IL2_I92F_L94F_L96F_R)
cagatcccttgaattcgaaaacaaatacgttg

SEQ ID NO: 388 - DNA, 39 bp, Artificial Sequence
  primer #175 (IL2_I92F_L94F_L96F_F)
gcaatatcaacgtatttgttttcgaatttaagggatctg

SEQ ID NO: 389 - DNA, 39 bp, Artificial Sequence
  primer #176 (IL2_I92F_L94F_L96F_R)
cagatcccttaaattcgaaaacaaatacgttgatattgc

SEQ ID NO: 390 - DNA, 39 bp, Artificial Sequence
  primer #177 (IL2_I92F_L94F_L96I_F)
gcaatatcaacgtatttgttttcgaaattaagggatctg

SEQ ID NO: 391 - DNA, 39 bp, Artificial Sequence
  primer #178 (IL2_I92F_L94F_L96I_R)
cagatcccttaatttcgaaaacaaatacgttgatattgc

SEQ ID NO: 392 - DNA, 39 bp, Artificial Sequence
  primer #179 (IL2_I92F_L94F_L96V_F)
gcaatatcaacgtatttgttttcgaagtaaagggatctg

SEQ ID NO: 393 - DNA, 39 bp, Artificial Sequence
  primer #180 (IL2_I92F_L94F_L96V_R)
cagatccctttacttcgaaaacaaatacgttgatattgc

SEQ ID NO: 394 - DNA, 33 bp, Artificial Sequence
  primer #181 (IL2_I92I_F)
gcaatatcaacgtaattgttctggaactaaagg

SEQ ID NO: 395 - DNA, 33 bp, Artificial Sequence
  primer #182 (IL2_I92I_R)
cctttagttccagaacaattacgttgatattgc

SEQ ID NO: 396 - DNA, 33 bp, Artificial Sequence
  primer #183 (IL2_I92L_F)
gcaatatcaacgtattagttctggaactaaagg

SEQ ID NO: 397 - DNA, 33 bp, Artificial Sequence
  primer #184 (IL2_I92L_R)
cctttagttccagaactaatacgttgatattgc

SEQ ID NO: 398 - DNA, 33 bp, Artificial Sequence
  primer #185 (IL2_I92W_F)
agcaatatcaacgtatgggttctggaactaaag

SEQ ID NO: 399 - DNA, 33 bp, Artificial Sequence
  primer #186 (IL2_I92W_R)
ctttagttccagaacccatacgttgatattgct

SEQ ID NO: 400 - DNA, 32 bp, Artificial Sequence
  primer #187 (IL2_I92Y_F)
gcaatatcaacgtatatgttctggaactaaag

SEQ ID NO: 401 - DNA, 32 bp, Artificial Sequence
  primer #188 (IL2_I92Y_R)
ctttagttccagaacatatacgttgatattgc

SEQ ID NO: 402 - DNA, 33 bp, Artificial Sequence
  primer #189 (IL2_L94F_L96F_F)
cgtaatagttttcgaatttaagggatctgaaac

SEQ ID NO: 403 - DNA, 33 bp, Artificial Sequence
  primer #190 (IL2_L94F_L96F_R)
gtttcagatcccttaaattcgaaaactattacg

SEQ ID NO: 404 - DNA, 33 bp, Artificial Sequence
  primer #191 (IL2_L94F_L96I_F)
cgtaatagttttcgaaattaagggatctgaaac

SEQ ID NO: 405 - DNA, 33 bp, Artificial Sequence
  primer #192 (IL2_L94F_L96I_R)
gtttcagatcccttaatttcgaaaactattacg

SEQ ID NO: 406 - DNA, 33 bp, Artificial Sequence
  primer #193 (IL2_L94F_L96V_F)
cgtaatagttttcgaagtaaagggatctgaaac

SEQ ID NO: 407 - DNA, 33 bp, Artificial Sequence
  primer #194 (IL2_L94F_L96V_R)
gtttcagatccctttacttcgaaaactattacg

SEQ ID NO: 408 - DNA, 30 bp, Artificial Sequence
  primer #195 (IL2_E95D_F)
gttctggacctaaagggatctgaaacaaca

SEQ ID NO: 409 - DNA, 30 bp, Artificial Sequence
  primer #196 (IL2_E95D_R)
tgttgtttcagatccctttaggtccagaac

SEQ ID NO: 410 - DNA, 33 bp, Artificial Sequence
  primer #197 (IL2_C125S_F)
agatggattacctttagtcaaagcatcatctca

SEQ ID NO: 411 - DNA, 33 bp, Artificial Sequence
  primer #198 (IL2_C125S_R)
tgagatgatgctttgactaaaggtaatccatct

SEQ ID NO: 412 - DNA, 34 bp, Artificial Sequence
  primer #199 (IL2_Q126T_F)
gatggattacctttagtacaagcatcatctcaac

SEQ ID NO: 413 - DNA, 34 bp, Artificial Sequence
  primer #200 (IL2_Q126T_R)
gttgagatgatgcttgtactaaaggtaatccatc

SEQ ID NO: 414 - DNA, 33 bp, Artificial Sequence
  primer #201 (IL2_desA1_F)
taagaatatacatatgcctacttcaagttctac

SEQ ID NO: 415 - DNA, 33 bp, Artificial Sequence
  primer #202 (IL2_desA1_R)
gtagaacttgaagtaggcatatgtatattctta

SEQ ID NO: 416 - DNA, 34 bp, Artificial Sequence
  primer #203 (IL2_NdeI_desA1_N-term)
cgccatatgcctacttcaagttctacaaagaaaa

SEQ ID NO: 417 - DNA, 34 bp, Artificial Sequence
  primer #204 (IL2_BHI_C-term)
cgggatcctcaagtcagtgttgagatgatgcttt